European Patent Application EP 4 159 861 A1, published April 5, 2023. Title: METHOD FOR PREPARING A PLASMID COMPRISING TYPE I POLYKETIDE SYNTHASE. Applicant: Spiber Inc. The sequence listing filed with the application follows.

SEQUENCE LISTING (31 sequences)

SEQ ID NO: 1 - DNA, 10638 bp, Artificial Sequence
  codon-optimized EryAI
atggccgacttatcgaaactgtcagattcgcgtaccgcccaacccggccgcattgtgcgcccttggccacttagtggttgtaacgaatctgcccttcgtgcccgcgcgcgccaactgcgtgcccacttagaccgctttccggacgccggcgtggaaggcgtgggtgcagcgctggcacatgatgaacaagcagatgcaggcccccatcgtgctgttgtggtggcaagctctactagcgaactgttagacggtctggcggccgtggcggatgggcgcccacatgcctcagtagttcgtggcgtagctcgcccgtcagcacctgttgttttcgtatttccgggtcaaggagcccaatgggcgggcatggccggtgagttgctgggtgagtcccgcgtgttcgcagcggcgatggatgcttgcgcacgtgccttcgaacccgtgacagattggaccctcgcgcaagtactggattcaccggaacaaagtcgccgcgtagaagtagtacagccggcgctgttcgcagtgcagacgagcctcgcagccttatggcgcagtttcggggtgacgccagacgccgtggttggccactccattggcgagctggcggcagcacacgtttgtggcgcagcgggtgcagccgatgcagctcgcgcagcggctctctggagtcgcgaaatgattccgttagtaggtaatggagacatggcagccgttgcgctgtctgcagacgaaattgagccccgcatcgcccgctgggacgacgatgttgttttagcaggggtcaacggcccgcgctccgttcttcttacgggctcgccggagccggtcgcacgtcgcgtgcaagaactttcggccgagggtgtgcgcgcacaggttattaatgtgagcatggcggcccattccgcgcaggttgatgacattgcggaaggcatgcgctcggccctggcatggtttgcaccgggtgggagcgaggtgccgttttacgccagtctgaccggtggtgccgtagacacccgtgagctggttgcggattactggcgtcgcagctttcgtctccccgtgcgttttgatgaggccattcgtagtgcacttgaagtgggcccggggacgtttgtagaggcatcaccccaccccgtgcttgccgcagcattacagcagaccctcgacgccgaaggctcgtcagccgcggtagtgccaacgttacaacgcggccaaggtgggatgcgccgtttcctgctcgctgccgcgcaagcgtttacgggcggcgtggcggtggactggaccgcggcgtacgatgacgttggggcggaacctggtagtctgccagagtttgccccagccgaagaagaggacgaaccggcagagagcggtgtggactggaacgcaccgccacacgtgctccgcgaacgtctccttgcggtcgtgaacggtgaaacggcggcattagctggtcgcgaggctgatgcagaggcaaccttccgcgaactcggcttggatagcgtcttagcggcccagttacgtgcgaaggtatcagccgccattggacgtgaggtcaatatcgcactgttatacgaccacccaacccctcgtgctctggctgaagcgctggcggcagggaccgaggttgcccaacgtgagacacgcgcacgtaccaacgaggcggcgcctggcgagccggtggccgtcgttgcgatggcctgtcgccttccgggcggtgtatccacaccggaagagttttgggagttgctctccgagggtcgtgatgccgttgcggggttaccgacagatcgcggctgggacctggactcgctgtttcatccggatccgactcgtagtggaaccgcgcatcagcgtggaggagggtttctgactgaggccacggcgttcgacccggccttcttcggtatgagcccgcgcgaagctcttgctgttgacccgcagcagcgcctgatgcttgagctctcttgggaagtgttggagcgcgcgggcattcccccgacctcacttcaagcttcacctacaggggtatttgttggcctgattccgcaagagtacggcccgcgtttagcggaaggcggagagggagttgagggctacctgatgaccgggacgacgacgagcgtggcgagtggccgcatcgcgtatacgctgggcttagagggccctgctatcagcgtagacaccgcgtgcagtagttcattggttgccgtacatttggcctgtcagagccttcgtcgcggtgagagctctttagcgatggccggtggggtgaccgtgatgcctacgcctgggatgctcgttgacttttcacgtatgaactctctggcacccgatggtcgttgtaaagcctttagcgcaggagctaacggttttggcatggccgagggtgcggggatgctcttgttagaacgcttatcggatgcgcgtcgtaatggtcatccagtactggcggttctgcgtggcaccgcggtaaattctgacggcgcctcaaacggcttgagtgcacctaatggtcgcgcgcaggtacgtgtgattcagcaagctctggcggaaagtggcttgggtccggccgacattgatgcggtggaagcgcatggaacaggtacgcgcctgggcgatccgattgaagcacgcgctctgtttgaagcctatggccgcgaccgtgaacaaccgttacacctcggcagcgtcaaatccaacctgggccacacccaggcggcggctggcgtcgcgggtgtcattaaaatggtcctcgctatgcgcgccggtacgctgcctcgtacgttacatgcttcggaacgttctaaagagatcgattggtcgtcgggcgcaatttctctgttagacgagccggaaccgtggccggcgggagctcgtccacgtcgtgcgggcgttagctcattcggcatctccggcacgaacgcccacgccatcatcgaagaagcgcctcaagttgtagagggcgaacgcgtcgaagcaggagatgttgttgcaccctgggttctctcagccagcagcgccgagggcttacgtgcgcaggcggcccgtcttgccgcgcatctgcgtgaacacccgggccaggacccacgcgatattgcgtatagtcttgcaactggacgcgcggccctgccacaccgcgccgcatttgcacccgtggatgaaagcgccgccctgcgcgtgcttgatggtctggccacagggaatgccgacggcgcggcagttggtaccagtcgcgcacagcaacgcgccgtgtttgtatttcctggtcagggttggcagtgggctggcatggccgtggatttgctggatacaagccctgtgttcgccgctgcattacgtgagtgtgcggacgcactggaaccgcaccttgactttgaagtaattccgttcctgcgtgccgaggcagcacgtcgtgaacaggatgcggcgttatctactgaacgtgtggatgtcgtgcagccagttatgttcgcggtgatggtatcgttagccagcatgtggcgcgcccacggggttgaaccggccgcagtgattggtcacagccaaggggaaatcgcagcagcttgcgttgccggcgcgttaagtctggacgacgcagcccgtgtggtagccttacgtagccgcgtgatcgccactatgccgggcaacaaagggatggcaagcattgcggcaccagcgggcgaggttcgtgcccgcattggagatcgcgtcgaaatcgcggcggtaaacgggccgcgtagtgtggttgtggccggtgactccgatgagttagatcgcctcgtggcatcctgcaccacggaatgtattcgcgcaaaacgtctcgcagttgactacgcgtcacattccagccatgtcgagactattcgtgacgcgctgcatgcagaattaggtgaagattttcatccgcttcccgggtttgtgccgttcttctccacggtaaccggccgctggacgcagcctgacgaacttgacgccgggtattggtatcgtaacctgcgtcgtaccgtgcgtttcgcggatgccgtacgtgcccttgcagagcaaggatatcgtacgttcttagaagtgagcgcacacccgattctcacagcggcgatcgaagagattggtgatggcagcggagcggacttgagcgcaattcattccttacgtcgtggcgacggctcattagccgattttggcgaggcgctgagccgcgcgtttgccgccggtgtcgccgtggattgggagtccgttcatcttggtaccggggcgcgtcgcgttccactgcctacctatccctttcaacgcgagcgtgtgtggttggaacctaaacctgtcgcgcgccgcagcacggaagtggatgaagtttcagcactgcgttatcgtattgaatggcgtcctaccggcgcgggcgaaccggcgcgccttgacggcacctggctggtagctaaatatgccggcacggcggatgagacgtcaacagcggcccgtgaagccctggagagcgcgggcgcccgtgttcgcgagcttgttgttgatgcccgttgtggccgtgacgaactcgccgaacgtctgcgcagtgtcggcgaggtagccggtgtactttcactgttagcggtggacgaagccgaaccggaagaagcgccgctcgcgctggccagtcttgcggatactctgtcactggttcaagccatggtgtcagcggaacttggttgtcctttatggactgttactgagagtgccgtagcgaccggtccctttgagcgcgtacgtaacgcggctcacggcgcactttggggagtgggtcgtgtcattgccttagagaacccggccgtctggggcggcctggttgacgttcccgccggctcggttgcggaacttgctcgccacttagcggcggtggttagtggtggagcgggtgaagatcaactggcgctccgtgcggatggagtgtacggccgccgctgggtgcgcgcggcggcccctgcgaccgatgatgaatggaaaccgaccggaaccgtgcttgtgacaggcggtaccggtggggtaggtggccagattgcacgctggctggcacgtcgtggggcgccgcatctgttactggtatcccgctccggaccggacgcagatggcgctggcgagctggttgcggaattggaagcacttggggcacgcacgaccgtagctgcgtgcgatgtgacggaccgtgaatcggtccgtgagcttctgggcggcatcggtgacgatgtacctctctcggccgttttccatgcggcagcaactctggacgacggtacggtggatactttaaccggcgaacgcatcgaacgtgcgagccgcgccaaagtgctgggtgcccgtaatttgcacgagcttacccgcgagcttgacttaactgcgttcgttttatttagtagcttcgcgagcgcctttggggccccgggcttgggtggatacgcgccgggtaacgcctatctggatggattagcccagcaacgccgttcagacggcttgccggcgacggcagtggcctggggcacctgggccggctccgggatggccgaaggtccggttgcggatcgcttccgccgtcacggcgtaattgaaatgcccccggaaaccgcgtgtcgcgctctgcaaaacgcactcgaccgtgccgaggtatgtccgatcgtaatcgatgtgcgttgggaccgtttcttactggcctataccgcacaacgcccgacgcgcctgttcgacgagatcgatgatgcgcgccgcgcggccccgcaggcggcggccgagcctcgtgttggagctttggccagtctgcctgcaccggagcgcgagaaagccctgttcgaactcgtgcgcagccatgctgcggcagtactgggccacgcgagcgccgagcgtgtccctgcggaccaagcattcgccgaacttggcgtggactcgttatcggcgcttgaactgcgtaatcgccttggcgcggccaccggcgtacgtctgccgacgacgaccgtgtttgaccatccggatgttcgcaccctggcggcccatctggcggccgaacttggtggtgccactggagccgaacaggcggcgccggccaccaccgcgccggtagatgagccgatcgcaattgttggcatggcgtgtcgccttccgggtgaagtcgactcgccggagcgtctttgggagttaatcacaagtgggcgtgattccgctgccgaagtacccgatgatcgcggctgggtgccagatgagctgatggcctctgacgcagcaggtacccgccgtgcgcacggtaactttatggcgggcgcaggagactttgatgctgcattctttggaatttctccacgtgaagcattggcaatggacccacaacaacgtcaagccttagagactacctgggaagcacttgaaagtgctggtattccgccagagacgttacgcggctcggacacaggcgtattcgtcggcatgagccatcaggggtacgccacaggccgtccgcgtccagaagatggtgttgatggctatctcttgaccggcaatacagccagcgtggcaagcgggcgcatcgcctatgtgctgggcctcgaaggaccggcgttaactgttgatactgcatgtagttcgtctctggtggctctgcacaccgcatgcggcagcttacgcgacggcgactgtggcttggcagttgcaggcggtgtgtcagtgatggccgggcctgaagttttcaccgaattttcgcgtcaaggtgccctttctcctgacggacgctgcaaaccctttagcgatgaggccgacggctttggtcttggtgaaggtagcgctttcgtcgtcctgcaacgtcttagtgatgcacgccgtgaaggccgccgcgtgttaggcgtggtggcgggcagtgctgtgaatcaggacggtgcatcgaacggattaagcgcgcccagcggagtggcgcagcaacgcgtcattcgtcgcgcatgggctcgtgcaggtattacaggtgcagatgtcgcggtggtcgaggcgcacggtacaggcacccgccttggtgaccctgtggaagcctcagcccttttggccacgtacggtaaaagccgtggctcgtctggcccggttttactcggatctgtgaaaagcaacattggacatgctcaggccgcagccggcgttgctggtgtgattaaagtcctgcttgggcttgagcgtggagtagtgccgcccatgctgtgccgtggcgagcgttccggtctgattgattggtctagcggtgagattgaacttgccgacggtgtccgcgagtggtcccctgcagccgacggggttcgtcgcgcgggagtaagtgcattcggtgtaagtggtaccaacgctcacgtgattattgcagaaccgccagaacccgagccggtcccgcaacctcgtcgcatgttaccggcgactggcgtcgtgcctgtcgtgctgtctgcccgtacaggggcggcactgcgcgcccaagctggacgcttagctgatcacttagccgcgcacccgggcattgctccagccgacgtcagctggaccatggctcgtgcacgccaacacttcgaagaacgcgccgccgtattggccgcggacaccgcagaggccgtgcatcgtttgcgcgccgttgccgacggagcagtcgttcctggcgtggtcacaggtagcgcctctgacggtggttcggttttcgttttccccggccagggcgcccaatgggaaggcatggcccgcgagctcctgccagtaccggtgttcgcagaaagtattgcggaatgcgatgctgtgctgagcgaagtggccggattttccgtctctgaagtactggagcctcgtccggatgcgccgtctctggagcgtgttgacgtagtgcaacctgtgcttttcgccgtgatggtgtcactggcccgcctgtggcgcgcatgtggcgcagtcccatctgccgtgattggccattcacagggcgagattgctgcagcagttgtagctggtgcgttgtccttagaggacggcatgcgcgttgttgcgcgccgctcgcgtgccgtccgcgctgtagcggggcgcggctccatgctgtcggtccgtggtgggcgctcagacgttgagaaactgttagccgatgacagctggaccggccgcctggaagtagccgccgtcaacggtcctgatgcagtggtcgtggccggcgacgcgcaggcagcgcgcgaatttctggagtactgcgaaggcgtaggcattcgcgcccgtgcaatcccggtggactatgcatcgcacacggctcatgtggaaccggttcgtgatgagttagtacaagccctcgcggggattacacctcgtcgcgcagaagtacctttcttctcgaccttgactggtgacttcctggacggcacggagcttgacgccggctactggtatcgcaatctgcgccatccggtcgaatttcactctgcagtccaagctttaacggatcaagggtacgcgacctttattgaggtgagtccgcatcctgtgctcgcatcaagcgtgcaggaaacccttgatgatgcagaatccgacgccgcagtacttggaaccctggagcgcgacgctggtgatgcggatcgctttctgactgcacttgcggatgcgcacacgcgcggagtcgcagtcgactgggaagcggtactgggacgcgcagggttggtggatcttcctggataccctttccaaggtaaacgcttctggctgctgccggatcgtacgactccgcgcgatgaattggatgggtggttctaccgcgtagattggacagaagttccgcgtagcgaacccgccgcgctgcgcggccgttggcttgtggttgtgccggaaggacacgaagaagatggctggacggtggaagtacgctcggcattagccgaggcaggagcggaaccagaggttacgcgtggagtgggtgggctggttggtgattgcgcaggggtcgtcagcctgctggccctcgaaggggacggcgccgttcaaacgctcgtactggtgcgcgaattagatgcggaaggcattgatgcgccactctggacggttactttcggtgcagttgatgcggggagcccggtcgcacgtcctgaccaggccaaactctggggtctgggccaagtggcgtcattagaacgtggcccgcgctggactggtctggttgacctgccgcacatgccagaccctgagcttcgtggacgcctgacggccgtccttgccggaagcgaggaccaagttgcggttcgcgctgacgccgtgcgtgcccgccgtctgtcaccggctcacgttacagcaacgtcagaatatgctgtcccgggcggcacgatcttagtgacaggcggcacggcaggattaggtgccgaggttgctcgctggttagctggccgcggggccgaacatttggcactggttagccgccgcgggcctgataccgaaggcgtaggtgacttaaccgccgagctgacacgcctgggtgcgcgcgtgagtgtgcatgcatgtgatgttagctcacgtgagccggtgcgcgagcttgttcatggcctgattgaacaaggcgatgtagttcgcggagttgtgcatgcagcaggtttaccccaacaagtggccatcaatgacatggatgaggcagcgtttgacgaagtagttgcagcgaaagcgggcggggccgtgcacctggacgaattatgctcagatgcggaactgtttctcttatttagctccggtgccggtgtatggggctctgcccgccagggagcgtatgcggcgggcaacgcctttctggacgcgttcgctcgccaccgccgtggtcgtggtttacccgcgactagcgtggcgtggggactctgggcggcgggcgggatgaccggcgacgaggaagccgtctcattcttgcgtgaacgtggagtccgtgcgatgccggtaccgcgcgccctggcggcgctcgaccgtgttctggcgagtggggaaactgcagtcgtggtaactgacgtcgactggccggcgttcgccgaatcatacaccgcggcacgcccgcgtcctctgttagatcgcattgtgaccaccgcaccatcagagcgtgcgggtgagccagaaacggaatcgcttcgcgatcgtctcgctggattaccacgcgctgagcgcaccgcggaactggtacgcttagtacgtactagtaccgcgaccgtcttgggccacgatgatccaaaggcggtccgcgccacgaccccgtttaaagaattaggcttcgatagcttagccgctgttcgtttacgcaacttactcaatgcagccaccggcctgcgtctgcctagtacgctggtattcgaccacccgaacgcgagtgccgtggctggtttcctggacgccgagcttggtactgaagtgcgtggcgaggctccatcggctctggccggacttgatgcactggaagcggcccttcctgaggtacctgccaccgaacgtgaagagctggtgcaacgcttagaacgtatgttagcggctttacgtccagtcgcacaggctgcagacgcaagcggtacaggtgcaaatccgagcggagatgatctgggtgaagcaggcgttgacgagctccttgaggccctcggccgcgagttagacggggactaa

SEQ ID NO: 2 - DNA, 10704 bp, Artificial Sequence
  codon-optimized EryAII
atgacagattcagagaaagttgcagagtacttgcgccgcgccacgcttgaccttcgtgccgcgcgccaacgcattcgtgagctggaaagcgatcccattgcgatcgtctcgatggcgtgtcgtctgccgggtggtgtgaacaccccacaacgtttatgggagctgctccgtgagggcggggaaaccttgtcgggctttcccaccgatcgtggctgggaccttgctcgtttgcatcacccggacccggataatccaggaacgtcttatgttgataagggcggtttcctggatgacgccgcaggatttgacgccgagttcttcggcgttagcccgcgtgaagccgccgccatggatccccaacaacgtttacttctcgaaacgagctgggaattagtggagaacgcgggtattgaccctcatagtctgcgcggaaccgcgacgggtgtgtttctgggcgtggcgaagttcgggtacggagaagatacagccgcggctgaagatgttgaaggctacagcgtgactggcgtcgcacccgcggttgcctctggtcgtattagctatacgatgggcctggaagggccgagcatcagcgtggacactgcgtgcagcagctcgctggtggcgttgcacctggccgttgagagtctgcgcaaaggtgagagtagtatggcggtagtgggtggtgccgccgtcatggcgacgcccggagtctttgtcgacttctcccgtcagcgcgcactcgccgcagatggacgtagtaaagcgtttggcgccggtgccgatggtttcgggttctcagagggtgtcactcttgtgttactggagcgtctttcagaggcacgtcgtaatggacacgaagttttagctgttgtgcgtggatcggcgttaaaccaggatggcgcatccaacggattgagcgcgccatcgggcccggcccaacgccgcgtaattcgccaagcgttagaatcgtgtggtcttgaacctggcgatgttgatgcggttgaggcccacggcaccggcactgctttaggcgacccgatcgaagcgaacgccctgctggacacctatggacgcgatcgcgatgcagatcgcccgctttggttaggctcagtcaagagtaatattggacacacccaggcagcagcgggtgttaccggcttacttaaggtggtcctggcattacgtaacggcgagctgccagccaccttacatgttgaggagcccacaccgcacgtcgattggtcatctggcggtgtggccctgttagccgggaaccagccgtggcgccgcggggagcgtacccgtcgtgcggcagtgtcagcatttggcatctcgggtaccaatgcccatgttatcgtagaagaggccccggaacgcgagcatcgtgaaaccactgcccacgatggtcgcccagtgccgttagtggtgagcgcgcgtagcacggcggcacttcgcgcccaagcggcacaaattgccgaactcttagaacgcccggacgcagatcttgctggcgttggattaggcctggccactacccgtgcgcgccatgaacaccgcgcggctgtcgtggcgtccacacgtgaagaagcggttcgcggtctgcgcgaaatcgcagccggtgcggccactgcggatgccgtagtggaaggcgttaccgaggtggacggtcgcaatgtggttttcctctttcctggtcagggctcgcagtgggcgggcatgggcgcagaactcctttcaagcagtcctgttttcgcaggaaagattcgtgcgtgcgacgaaagcatggcgccgatgcaagattggaaggtttctgatgtgttacgccaagcaccaggagcgccaggcctcgaccgcgtagacgtagttcaacccgtgctgtttgctgtcatggtgtcgttagctgagctttggcgctcatacggcgtggagccggcggctgtcgtgggccattctcaaggtgaaattgcagcggcccacgtggcaggagcactgaccttggaagatgcggcaaaactcgtcgtgggtcgcagccgcctgatgcgctcattgtccggagagggcggcatggcggcggtggcgcttggtgaagcggcggtgcgtgagcgtctccgtccgtggcaagatcgcctgtcagtagctgcagttaatggccctcgcagcgttgtagtaagtggcgagccgggtgcgcttcgcgccttttcagaggactgtgcggccgagggcatccgcgtccgtgacatcgacgtcgattatgccagccattcacctcagatcgagcgcgtccgtgaagagctgctggaaaccactggagacattgccccgcgccccgcgcgcgtgacgtttcattcaactgtggaatcccgctcgatggacggcaccgaactggatgcccgctactggtaccgcaatctgcgtgagacggtgcgctttgcggacgcggtgactcgtttggccgagagcggttatgatgcgtttatcgaggtttctccgcacccggtggttgtgcaggccgtggaagaggctgtggaagaggcggatggggcggaagatgccgtggttgttggatctctgcatcgtgacggtggcgatctgagcgcgttcttacgtagcatggccaccgcccacgtttcaggggtcgacatccgttgggacgtagcattgccgggtgctgcgccgttcgcactgccgacgtacccgttccaacgcaaacgctattggcttcagcctgcggcaccggcggccgccagcgatgagcttgcgtaccgtgtgagctggacccctattgaaaagccggaatctggcaacctggacggcgattggctcgttgttacgccgctgattagcccagagtggacagaaatgttatgtgaagccatcaatgccaatggcggccgcgccttacgctgtgaggtggacaccagcgcgtcccgtactgaaatggctcaagccgtggcccaggccggtaccggcttccgtggagttctgtcattattaagcagtgatgagagcgcctgtcgtccgggcgtgccggcgggcgccgtagggcttctcactttggtccaagccctcggcgacgcaggcgtcgatgcgcccgtttggtgtctgacccaaggagccgttcgtaccccggcagatgacgatctggcccgcccggcccagacaaccgcacatggattcgcccaagttgccggcctcgaattaccgggccgttggggtggcgtcgttgatcttccggagagcgtggacgatgcggcactgcgtttattagtggctgtgttgcgcggtggcggccgcgcagaggaccacctggccgtacgtgatggccgtttgcatggccgccgcgtcgtacgtgctagcctgccgcagagcgggtcacgttcttggactccccacggcactgtattggtcactggggctgcttcgcccgtcggtgaccaactcgtgcgttggctcgccgaccgtggcgctgaacgtttagtccttgcaggcgcgtgcccgggagacgatctgctggccgccgtggaagaagctggcgcctcagcagtagtgtgtgcccaagacgccgcggccctgcgcgaagcgctcggcgatgaacccgttaccgcccttgtacacgcgggtaccttgaccaattttggtagcatctcagaggtggcgccggaagaatttgcggaaaccattgcggcgaaaaccgccctcttagccgtactggatgaagtccttggtgaccgtgcagtcgagcgtgaagtgtactgttcgtctgtggcgggtatttggggcggtgcgggtatggcggcgtacgcggcgggtagtgcgtacctcgacgcattagctgagcatcaccgtgctcgtggtcgtagctgcacgtcagtggcatggacgccgtgggcattacccggcggcgcggtggacgacggttatctccgtgagcgcggcctgcgcagcttgagcgctgatcgcgcgatgcgtacctgggagcgtgtcttggcagcgggtcccgttagcgtggcggtcgccgacgtcgattggccggtactgagcgaaggattcgcagcgacgcgcccgaccgccttattcgccgaattagccggccgcggcggacaagctgaagccgagcccgatagtggccccactggcgagccggcgcagcgcttggcgggcctctcacctgacgagcagcaggagaacttacttgagttagtcgcaaatgccgtggcagaggttttaggccatgagtcggcagccgaaatcaatgttcgtcgcgcgttctctgagcttggattggattctctgaatgctatggctcttcgtaaacgtttatctgccagcaccggattacgccttcctgcgagcttggttttcgaccacccgacagttactgccctggcgcagcacttacgcgcccgtcttgtcggtgacgcggatcaagctgcggtacgcgtagttggtgcagcggacgaatccgaaccgatcgctattgttggtatcggttgtcgttttccgggcggcattggatcgcccgagcaattatggcgcgttcttgctgagggtgcgaatctgacaaccggtttcccggctgaccgcgggtgggatatcggccgtttatatcatcctgatccggataatccgggcacatcctacgttgataagggcggcttccttacggatgccgcagattttgacccggggttcttcggtattacccctcgcgaggcgctggccatggatccgcagcagcgccttatgcttgagacggcctgggaagccgtagagcgtgcaggcatcgaccccgacgccttacgcggaacggacacaggagttttcgtgggcatgaacggacaatcttatatgcaattacttgcgggtgaggcggaacgcgtcgacggctaccagggcttgggtaacagcgcgagcgtcctcagcggccgcattgcctacacgttcggttgggaaggtcctgcgttaacagtggatactgcatgttctagcagtttggtgggtattcatttagcgatgcaagcccttcgtcgcggcgaatgctcactcgctttggcgggtggcgtaacggtcatgtctgacccgtacaccttcgttgatttcagcacgcagcgtggccttgcgagtgacggtcgctgtaaggccttcagtgcgcgtgcagacggtttcgccttatcagagggtgtcgcggccttagtgttggagcccctcagtcgtgcgcgtgctaatggccaccaagtgcttgccgtcttgcgcggcagcgcggtcaatcaggacggtgccagcaacgggctggcggcccctaatggtccgagccaggaacgtgtgattcgccaagccttagccgcgagcggagtgccggcggcagatgtggacgtggtagaggcccacggtacaggcacagaactgggtgacccgattgaggccggagcgttgattgccacgtatgggcaggaccgcgatcgtccactgcgtctgggaagcgtgaaaaccaatattggccatacgcaagccgctgcaggggcggctggtgtcatcaaagtcgtgctcgcaatgcgccacggtatgttgccacgctcgcttcacgcagatgagttaagccctcatattgactgggaatctggcgccgtggaagtgctccgtgaggaagttccgtggccggccggggagcgtccacgccgcgcaggcgttagctcgtttggcgttagcggaactaatgcccatgtgattgttgaagaagccccggcggaacaagaggccgcccgcaccgaacgcggtccgctgccgtttgtgctctcgggccgctccgaggcggttgtcgcggcgcaggcacgtgccttagccgaacatctgcgtgatacacctgagttaggcctgactgatgcggcctggacgctggccacgggtcgtgcccgttttgacgtacgcgccgcggttttaggcgacgaccgtgcgggtgtgtgtgccgagttagatgccttagcggaagggcgtccctcagcggatgccgtagcgccggtcacttccgccccgcgcaaacctgtactcgtctttccgggtcagggtgcgcaatgggtcggtatggcccgtgatctgctggagagtagcgaagttttcgcggagtccatgagccgttgcgcagaggccctgtcaccccataccgattggaagctcttggatgttgttcgcggtgatggcggaccggatcctcacgagcgtgtcgatgtgttacagccggtgctgttcagcatcatggtttctcttgcagagctgtggcgcgcgcacggcgtaaccccggcagcggtcgtaggtcactcacaaggcgaaatcgctgcggctcatgtagcgggcgcgcttagtcttgaggccgcagccaaagtggtggcgctccgctcccaggtattgcgtgaactggacgatcagggtggcatggtgtcggtgggcgcaagccgtgacgaactggaaaccgtgcttgcgcgttgggatgggcgtgtcgccgtggcagcggtcaacgggccgggtacctcggtggtcgccgggccaacggccgaattggatgagttcttcgccgaagccgaggctcgcgaaatgaagccccgtcgtatcgccgtacgctacgccagtcattcgccagaggtagcccgtattgaggaccgtcttgcagcagagctgggtacaatcaccgcggtccgtggttcagtgccgctgcatagcactgtaaccggggaagtaatcgatacctcagcgatggacgcgtcctattggtatcgtaacttacgccgcccggttttattcgagcaagcagttcgtggactcgttgagcagggcttcgacaccttcgtcgaggtcagtcctcatcccgtgctcttgatggctgtagaagaaaccgcggagcacgcgggtgccgaggtaacttgtgtacccacattacgtcgtgagcaaagcggccctcatgagttcttacgtaacttattacgtgcgcacgtgcacggagttggcgccgatcttcgtccagccgttgctggtggccgccccgccgaacttcctacatatccatttgaacatcaacgcttttggccgcgcccgcatcgccctgcggacgtgagcgcattgggtgtacgcggggccgagcatccgttgctgctggctgcggtagatgtcccaggccatggcggtgcggtgttcacgggccgtctgagtacagacgagcaaccgtggctcgctgagcatgtggtaggcggccgcaccttagttccgggttctgtgctggttgacctggcactcgcagcgggtgaagatgtaggtttacctgtgttggaagagttggtgcttcagcgcccgttagtgttagcaggggccggggcgcttctccgcatgtcggtgggagcccccgacgaaagcggacgtcgcacaatcgacgttcatgcggcggaagatgtagcggacttagctgatgcgcaatggtcacaacacgcaacgggcacgctggcccaaggcgtggccgcgggtccgcgtgacaccgaacagtggcccccggaagatgcggtgcgcatcccgcttgacgatcactatgacggactcgcggaacagggctatgaatacggaccttcgttccaagccttacgcgcggcgtggcgcaaggatgatagtgtctatgcagaggtttcgattgcggcagacgaagaaggttatgccttccatccggtccttttggatgcggttgcccaaaccttgtcgttaggggctttaggcgagccgggtggcggcaaattgccgtttgcatggaacactgtgacactccacgcgtccggggctactagtgttcgtgtggtggcgacgccagcgggcgcggacgcaatggcgctccgcgtgacagaccccgcagggcatctggtcgcgacggtcgattcattggtggtgcgcagcaccggtgagaaatgggaacagcccgagccgcgtggcggtgagggcgaattacatgcactggactgggtgcgtctcgcggaaccggggtcgaccggacgcgttgttgcagcggacgccagtgatttagacgcagtccttcgcagtggagagccggagccggatgccgtgctggtacgctacgaaccagagggtgatgacccgcgcgcagccgctcgccacggcgtattatgggcagccgcgttggtccgccgctggcttgaacaggaagagttaccgggcgccactctggttatcgcgactagcggcgcggtcacagtctctgatgacgactcggtgccggagccgggcgcggcggccatgtggggcgtgatccgttgtgcacaagcggagtcaccggatcgctttgttctgctcgatacagatgccgagcccggaatgctgccggcggtgccggacaatccccaactggcgttgcgtggtgacgatgtatttgtgccgcgtttatccccgctcgcaccttcggcactgactttaccggcgggtacccagcgtcttgtacccggagatggggccattgattccgtagccttcgagccggcgcctgacgttgagcaaccgctccgtgccggcgaagtgcgtgtagatgtccgcgcgaccggtgttaacttccgcgacgttcttcttgcactgggcatgtacccgcagaaggcagatatgggaacagaggccgcgggcgtagtaacggcagttggcccggacgtggacgctttcgcccccggcgatcgtgtactgggacttttccaaggcgcctttgcgccgattgcggtaacggaccatcgcctgttggcacgtgttccagacggatggagcgacgcagacgctgctgcggtacctattgcgtacaccacagcgcattacgccctgcacgatttagccggccttcgtgcaggccagtcagtgcttatccatgccgcggccggtggcgttggtatggctgccgtggcccttgcgcgccgtgccggcgcggaagttttagccacagcgggtccagccaaacatggcacgttacgtgcgctgggcttagacgatgaacacattgcgagttctcgcgagacaggttttgcgcgtaaattccgtgagcgtaccggtggacgcggcgtcgatgtagtgttgaacagtttaaccggcgaactcttagacgagagcgccgaccttcttgcagaggacggtgtattcgtagaaatgggtaaaaccgatctgcgcgacgcaggcgatttccgcggccgttacgcgccgtttgacttgggcgaggcgggcgatgaccgcctcggcgaaattcttcgcgaagtggtgggcctgcttggcgctggagaactggatcgtctgccggtttcagcctgggaattaggcagcgcacccgcagcgcttcagcacatgagccgcggacgccacgtcggcaaactggtcttgacccaaccggctccggtagatccagacggcactgtgctgattactggcggaacaggaactctgggtcgcttactggcccgccacttggtcacggaacacggcgtgcgtcatctgcttctggtttcacgtcgcggcgcagacgcccctgggagtgatgaacttcgcgcagaaatcgaggacttaggtgcgagcgcagaaatcgcagcgtgcgatactgcagatcgcgacgccctgtcggcgcttcttgatggcctgcctcgtcccttaaccggagtcgtgcatgcagccggtgtcctggccgatggcctggtcacaagcatcgatgaaccggcggtcgagcaagtacttcgcgcaaaagtggatgcggcatggaatctgcacgagttaaccgccaatacgggcctctccttctttgttctgttcagttccgcggcgtcggttctcgcgggaccgggacagggtgtatatgcagccgctaacgaaagcctgaatgccctggccgcgcttcgccgcacacgtgggttaccggccaaagcgctcggatggggcttgtgggcacaggcgtcggagatgacgtccggccttggcgaccgcatcgcgcgtactggtgtagcggcgctgccaacggaacgcgccctggccttgtttgatagcgcgttacgtcgcggcggtgaagtagttttccctctgtcaattaaccgcagcgcattgcgtcgcgcggaattcgtgccggaagtgctgcgtggtatggtccgcgcgaagttgcgcgcggcgggccaagccgaagcggcgggcccgaacgtcgtggatcgcctcgccggccgttccgaatcagaccaggtcgcgggtcttgcggagcttgtgcgttcacatgcagcggctgtctccggctatggcagcgcggatcaattaccggagcgtaaagcatttaaggaccttggctttgacagccttgcggccgtagagctgcgcaatcgtctgggcactgcgaccggtgtacgtttgccttcaacgctggtgtttgaccacccgacgcccctcgctgtagcggagcaccttcgcgaccgcctcttcgcagcgagtccggcggttgacattggtgaccgtctcgacgaacttgaaaaggcattagaggctctcagcgcagaagatgggcacgatgatgttggtcaacgcctggagagcctgctccgtcgctggaattcccgccgtgctgatgcaccgagcaccagcgcgatctctgaagatgcatctgacgatgaactgtttagcatgttggaccagcgttttggcggcggcgaagatctctaa

SEQ ID NO: 3 - DNA, 9516 bp, Artificial Sequence
  codon-optimized EryAIII
atgagtggagacaatggcatgacggaagagaaactgcgtcgttatctgaaacgtactgtcactgaattggatagtgtgacagcgcgcctgcgtgaagtcgaacaccgcgccggcgaaccgattgcgattgtggggatggcatgccgtttcccaggtgacgtagattcgccggagagtttctgggagtttgtaagcggcggcggtgacgcgattgcggaagcgcctgcggatcgtggctgggagcctgatccggatgcacgtcttggtggaatgctggcggcggcaggggattttgatgccggcttcttcggcattagcccacgtgaagcattggccatggatccgcaacaacgtattatgttggaaatttcgtgggaagcgctggagcgcgctggtcatgaccctgtgagtttgcgcgggagtgcgaccggggtgttcaccggagtggggaccgtggactatggcccccgtccagatgaagcacctgacgaagttttaggttatgtgggcacgggaactgctagcagtgtagcctcggggcgcgtggcgtattgcctgggacttgagggcccagccatgactgtagatacagcctgcagcagtggcttaactgctctgcaccttgcaatggagagtttacgccgcgatgaatgtggtcttgcgttagcaggcggtgttactgttatgtctagtccaggcgcgttcacggaatttcgttcgcagggtggactcgcggccgacggccgttgcaaaccattttcgaaagccgcggatggtttcggcttagccgaaggcgcgggtgtccttgtactgcagcgtctgagcgctgcgcgtcgcgagggtcgcccggtattggcagtcctgcgcggtagcgcggtaaaccaagatggagcatcgaatggtcttacggcgccgtcaggcccggcccagcagcgtgttatccgtcgtgctctggaaaatgcgggcgtccgcgcaggcgatgtggattatgtcgaagctcacggaacgggcacgcgcttaggcgaccccatcgaggttcacgcgctcttatctacttatggcgccgagcgcgatccggatgacccgctttggatcggctccgtgaagagcaacatcggtcacacccaggcggctgcgggtgtggccggtgttatgaaggcagtgttagcgctgcgccatggcgagatgcctcgcacgctgcatttcgacgaaccgtcaccgcagatcgagtgggacttaggtgccgtttctgtggtgtcacaagcgcgcagctggccagcgggcgagcgcccgcgccgcgcaggagtgtcatcttttggtatctctggcactaacgcacacgtcatcgtggaagaggcgccggaagcagatgagccggaacccgctccggacagtggcccagttccacttgtgctcagcgggcgcgacgagcaagcaatgcgtgctcaagcgggccgtctggcggaccacctggcgcgtgaaccacgcaactcgctgcgtgatacgggatttacattagcaacccgccgcagcgcgtgggagcatcgcgcagtcgttgtgggagatcgcgacgatgccctggcgggtttgcgcgctgttgctgatggccgtatcgccgatcgcaccgcgaccggtcaggctcgcacccgtcgcggcgttgccatggtgtttccgggtcaaggtgcgcagtggcaagggatggcgcgcgacctgcttcgtgagagccaggtgtttgccgattcaattcgtgactgcgagcgtgctttagctccacatgtcgactggtcattaacggacttgctctctggcgcccgcccgctggatcgcgtggacgtggtgcagcctgcgctctttgcagtgatggtgtcattagcggccttatggcgttctcacggggtcgagcctgccgccgttgtaggccattcgcaaggtgagattgcggctgcccacgtagcgggtgcacttacgttggaagatgctgctaaacttgttgcagttcgttcgcgtgtgttacgtcgtttaggcggccagggcgggatggcaagcttcggcctcggtaccgaacaagcggccgagcgtatcggccgctttgcgggtgccttatctattgcctcggttaatggaccgcgttcggtggtggtagccggagagagcggcccgctggacgaattaatcgccgagtgtgaggctgagggcattaccgcgcgtcgtatcccggtggattacgcctcgcattcaccgcaggtagagagcctgcgcgaagagctcttaacggagttagccggtatttcaccggtttccgctgacgtagccttatattcaacgaccacaggccagcctattgatacagcaacaatggacaccgcctattggtacgcgaacttacgcgagcaagtgcgcttccaagatgcgacccgccaattagcagaggcaggctttgacgctttcgttgaggtaagtccgcacccggttttgaccgtgggaattgaggccaccttagacagcgcactgccggcagacgcgggtgcatgtgtcgtgggcactctgcgccgcgaccgcggcggtttagccgattttcacacagccctgggcgaagcctatgcccagggtgtagaagttgattggtcgcctgcgtttgcagacgcgcgccctgtggaactgccggtttaccctttccagcgccaacgttattggcttccgattccaactggtggccgcgcgcgcgatgaggacgatgactggcgctaccaggtggtttggcgcgaggccgaatgggaatcagcatctctggcgggtcgcgttctgttagtaaccggtccgggtgtcccgtccgaactgtcggatgcgatccgctctgggctcgaacagtcaggagcgaccgtgttaacctgtgacgtggaaagccgtagtacgattggtaccgctcttgaagccgcggatacagatgccctgagcaccgtagtaagcctgctttcgcgcgatggcgaagccgtggatccatcgctggacgcgttagctctcgtgcaagcgttgggcgctgcgggagtagaggccccgttatgggtgttgacccgtaacgcggtgcaggttgcggatggggaattagtggacccggcgcaagcaatggttggcggtcttggtcgcgttgttggaatcgaacaacctggccgctggggtggtttagtagacttagtcgacgcggatgccgcaagcattcgtagccttgcggcagtactggcggaccctcgtggtgaagagcaagtcgctattcgtgcagacggtattaaagttgcccgtctggtgccggcccctgcccgcgccgcacgtacgcgctggagccctcgcggaaccgtgttagtaaccggtggcaccggtggtatcggcgcccacgtggcgcgctggttagcgcgttcgggtgccgagcatttagtgctgttgggccgccgcggcgctgatgcccctggggcttcagaactgcgtgaagaacttactgccttggggaccggtgttaccatcgcagcctgcgatgtcgcggatcgcgcgcgcttagaagctgttttagccgcggaacgtgcggaaggccgtactgtgagtgcggtcatgcatgccgcaggcgtttctacgtctacaccccttgatgacctcaccgaggcggaattcaccgagatcgccgatgtgaaggtccgcggcactgtgaacctggatgaactttgcccggacctggacgcgtttgtgttattctccagcaacgcgggcgtatggggctctccgggcctggcgagctacgcggctgcgaacgctttcctggacggttttgcccgtcgtcgtcgttcggaaggggcccctgtgacttcgattgcatggggcctgtgggcgggacagaatatggcgggcgacgagggcggagagtacttacgtagccagggcctgcgcgctatggacccggaccgcgcagtagaagaattacatattactctggatcatggccagacgagcgtaagtgtggtggacatggatcgccgccgcttcgttgaactctttacagcggcccgtcatcgtccgcttttcgatgaaatcgccggagcacgcgcggaagcccgtcagtcagaagaaggtcctgccctcgcacagcgtttagcggcactgagcacagcggagcgccgcgagcacttggcgcacctgatccgcgctgaggtggccgctgtgctgggacatggggatgacgcggcaattgatcgcgatcgtgctttccgtgacctcggctttgacagcatgaccgcggtggacttacgcaatcgccttgcggccgtcacgggtgttcgcgaggcggcgaccgtggtatttgatcacccgacgatcactcgcctcgcagaccactatcttgaacgcctggtcggcgcagccgaggcggagcaggcgcctgcgttggtgcgcgaagttcccaaagatgccgatgacccgattgcaattgtgggaatggcctgccgctttccgggcggtgtgcataatccgggtgaactgtgggagtttatcgtgggcggcggcgacgccgtcactgaaatgcctaccgatcgtggctgggacttagacgcgttattcgatccagatccgcagcgccacggtaccagctattcccgtcacggcgcattcttagatggcgcagccgactttgacgcggcgttctttggtatctccccgcgcgaagcgctggccatggatccacaacaacgccaggtgctggagacaacatgggaactgttcgaaaatgcaggaattgatccgcatagtctgcgcggtagtgataccggcgtgtttcttggtgccgcctaccagggatacggtcaagacgcggttgtccccgaggacagcgaaggttatctgctcactggtaattcatcggccgtcgtttcgggtcgcgtggcgtatgttctcggtttagagggccctgccgtaaccgtagacactgcctgttcgtcgagtttggttgccctgcactcggcatgcggttctttacgtgatggtgattgtggcctcgctgtagctggtggcgttagcgtaatggcggggcccgaggtattcacggaatttagccgtcagggtgggctggcggtggacggacgttgtaaggctttctcagcagaggcagatggctttgggtttgcggaaggagtggccgtcgtattattgcagcgcttatcggacgctcgtcgtgcaggtcgccaggttctgggcgtggtggccgggtcggcgatcaatcaagatggtgcgtcaaatggccttgcggccccttcaggagtcgctcagcaacgcgtgattcgcaaggcgtgggctcgcgcgggcattactggcgcagacgttgcagtggtggaagcccacggtacaggcacccgccttggcgatccagttgaggcgtcagccctgctggccacctacggcaagtcgcgtggtagtagcggcccggtactcctgggtagcgttaaatccaatatcggtcatgcacaagccgcggccggtgttgcaggggtaatcaaggtggtcctgggattaaaccgtggactggtgccgccaatgctgtgtcgcggtgagcgttccccgctgattgagtggtcgtccggcggtgtcgagctggccgaggcagtttctccgtggccgccggcggcagacggagttcgtcgtgcgggtgtttcagccttcggggtgtcaggcactaatgcacatgtcattattgcagagccgccggaaccggagccgttaccggaaccgggtccggtaggtgttttggcggcggcaaactctgtacctgtgttacttagcgcccgtaccgagacggcgttggccgcccaagcgcgcctgctggaatctgccgtagatgattcggtgccgctcacggcgctggcgtcggctcttgcgaccggtcgcgcccaccttccgcgtcgtgccgcacttttggcgggcgatcatgaacagctgcgtggtcaattacgcgctgtcgctgaaggcgttgcggcacctggtgcaaccaccggcaccgcatctgccggtggagtggtctttgttttccctgggcaaggcgcacagtgggaaggcatggcccgcggtctgcttagcgttcccgtgttcgccgaatctattgccgagtgcgatgcggtcctgagtgaggtcgcgggattttccgcgtcagaagtgctggagcaacgccccgatgcgcccagcctggaacgtgtggacgtagtacagccagtgttattctccgtgatggtttcgttagcgcgcttgtggggcgcttgcggagtcagtccgagcgctgtgatcggacacagccagggtgaaatcgccgccgccgtggtagccggcgtgttgtcattagaggacggagttcgtgttgtggcattgcgcgcgaaggcactgcgcgctctcgcgggtaaaggcggcatggtgtccctcgcagcgccaggtgagcgtgcacgcgcgcttattgccccttgggaagatcgtatcagtgtagctgccgtaaattccccatcgtcggttgttgtttcaggtgatcctgaggcgctggcggaacttgtcgcgcgctgtgaagatgagggtgttcgcgccaagacactgccagttgattacgctagccatagtcgtcatgttgaagagattcgtgagacgattctggccgacttggatgggattagcgcccgccgcgcggccatccctctttacagcacgctgcacggcgaacgtcgcgacggcgcggacatgggcccgcgctattggtacgataatcttcgtagtcaggtccgctttgatgaggccgtgtccgcggcagttgcagatggccacgctacatttgttgagatgtctccacatcctgtgctcactgcggcggttcaggaaattgcggcagacgcggtagctattggtagccttcatcgcgatacagctgaagaacatctgattgcagaactggcgcgcgcccatgtccatggcgtggccgtggactggcgtaacgtgttccccgcggccccgcccgttgcgctgccgaactacccattcgagccgcaacgctactggcttgcccctgaagttagtgaccagcttgcggattcccgctaccgtgtggactggcgtcctttagccacgaccccggtggatttggaaggcggattccttgtacatggctccgccccggaatcgttgacctcggcagtcgagaaagccggcggtcgtgtggtccccgtggcatcagcagatcgcgaagccttagccgcagcccttcgtgaggttccaggtgaagtggccggggtgctgagtgtgcacaccggtgcggcgacccacttagccttgcatcaatccttgggagaggctggtgttcgtgcgccgctgtggcttgtcacatctcgtgccgtcgctttgggtgaaagtgagccggtggatccggaacaggcaatggtttggggccttggccgtgtgatgggcttagaaacaccggagcgctggggcggcttggttgaccttccggcggagcctgctccaggcgatggggaagcttttgttgcctgcctcggggccgacgggcacgaagatcaggtggctattcgtgatcacgcacgctacggccgtcgtttagtgcgtgcgccgctgggaacacgtgagtcgtcgtgggagccggccggcacggcgctggttacgggtggcaccggggcgctgggcggtcatgtcgcacgccacctggcacgctgtggagtggaagatttagtgttggtcagccgtcgtggcgttgacgcaccgggcgctgcagaactggaagcggagctggtggccctgggagcgaaaacgacaattacagcttgtgacgtcgcagaccgcgagcaattgtcgaagttgctggaagagcttcgtggtcaaggccgtcccgtgcgcactgttgtacatacagcgggcgtgcccgagtcccgtccgctgcacgagattggtgagctcgaaagtgtatgcgcggccaaagtaaccggcgcgcgcttgcttgatgaactctgcccggacgccgaaacctttgttctgttctcgtcgggagctggggtgtggggctcggctaatctgggcgcgtactccgcggcgaacgcttatttagatgcgttggcgcaccgtcgccgtgcggaaggtcgcgcggcaacgtcggtggcctggggtgcgtgggcaggcgaaggtatggccaccggtgatttagaaggcctcactcgccgtggcttgcgcccgatggctcccgagcgcgcgatccgcgccctgcatcaagcactggataatggggatacctgtgttagtatcgcggatgttgactgggaacgcttcgcagtcggcttcacggcagctcgtccgcgtccgctcctcgatgaattagtgactcccgccgtgggagccgttccggccgttcaagcagcgcctgcacgtgaaatgactagccaagagcttttagagtttacgcatagccatgtggctgccattttgggacatagttctcccgatgcagtcgggcaagatcaaccgtttaccgaattaggctttgactcgttgacagcagtggggcttcgcaaccaactccagcaggcaacgggcttggcccttccagcaacccttgtctttgagcacccgacggtgcgtcgcttagccgaccacattggtcagcagttggactctggtacgcctgcgcgtgaagcatcgagcgctctgcgtgatggctaccgccaagccggggtttccggtcgtgtacgctcgtacctggacttattggcgggcttgagcgactttcgtgagcacttcgacggttcggacgggtttagccttgacctggtcgacatggcggacggacccggtgaagttaccgtaatctgttgcgcgggaacagctgcgatttcaggccctcacgagtttacgcgtttggccggtgctttacgcggaatcgccccagtacgcgccgttccgcagccgggttatgaggaaggggaaccgcttccgtcgtccatggcagcagtggcagcagtgcaggccgatgcagtgatccgcacccaaggcgataaaccttttgttgtagcgggccattctgccggcgccttaatggcgtatgcccttgcgacagaactcttagatcgcggccacccgccgcgtggagtagtcttgattgacgtctacccgccagggcatcaagacgccatgaacgcgtggttagaggaactcaccgcgacgttatttgaccgtgaaacggtgcgtatggatgatacgcgcttgaccgcacttggcgcctatgatcgcctgaccggccaatggcgtccgcgtgagacaggtttgcctactttgcttgtgtcggccggcgagcccatgggtccctggcccgacgattcgtggaaaccgacctggccgttcgaacatgacaccgtggccgtgcctggggaccattttaccatggtgcaggaacacgcagatgctatcgcccgccacattgatgcgtggcttggcggtggtaatagctaa

SEQ ID NO: 4 - DNA, 1151 bp, Artificial Sequence
  DNA fragment
tagggtctcactcagcagaggcagatggctttgggtttgcggaaggagtggccgtcgtattattgcagcgcttatcggacgctcgtcgtgcaggtcgccaggttctgggcgtggtggccgggtcggcgatcaatcaagatggtgcgtcaaatggccttgcggccccttcaggagtcgctcagcaacgcgtgattcgcaaggcgtgggctcgcgcgggcattactggcgcagacgttgcagtggtggaagcccacggtacaggcacccgccttggcgatccagttgaggcgtcagccctgctggccacctacggcaagtcgcgtggtagtagcggcccggtactcctgggtagcgttaaatccaatatcggtcatgcacaagccgcggccggtgttgcaggggtaatcaaggtggtcctgggattaaaccgtggactggtgccgccaatgctgtgtcgcggtgagcgttccccgctgattgagtggtcgtccggcggtgtcgagctggccgaggcagtttctccgtggccgccggcggcagacggagttcgtcgtgcgggtgtttcagccttcggggtgtcaggcactaatgcacatgtcattattgcagagccgccggaaccggagccgttaccggaaccgggtccggtaggtgttttggcggcggcaaactctgtacctgtgttacttagcgcccgtaccgagacggcgttggccgcccaagcgcgcctgctggaatctgccgtagatgattcggtgccgctcacggcgctggcgtcggctcttgcgaccggtcgcgcccaccttccgcgtcgtgccgcacttttggcgggcgatcatgaacagctgcgtggtcaattacgcgctgtcgctgaaggcgttgcggcacctggtgcaaccaccggcaccgcatctgccggtggagtggtctttgttttccctgggcaaggcgcacagtgggaaggcatggcccgcggtctgcttagcgttcccgtgttcgccgaatctattgccgagtgcgatgcggtcctgagtgaggtcgcgggattttccgcgtcagaagtgctggagcaacgccccgatgcgcccagcctggaacgtgtggacgtagtacagccagtgttattctccgtgatggtttcagagacccta

SEQ ID NO: 5 - DNA, 1139 bp, Artificial Sequence
  DNA fragment
tagggtctcatttcgttagcgcgcttgtggggcgcttgcggagtcagtccgagcgctgtgatcggacacagccagggtgaaatcgccgccgccgtggtagccggcgtgttgtcattagaggacggagttcgtgttgtggcattgcgcgcgaaggcactgcgcgctctcgcgggtaaaggcggcatggtgtccctcgcagcgccaggtgagcgtgcacgcgcgcttattgccccttgggaagatcgtatcagtgtagctgccgtaaattccccatcgtcggttgttgtttcaggtgatcctgaggcgctggcggaacttgtcgcgcgctgtgaagatgagggtgttcgcgccaagacactgccagttgattacgctagccatagtcgtcatgttgaagagattcgtgagacgattctggccgacttggatgggattagcgcccgccgcgcggccatccctctttacagcacgctgcacggcgaacgtcgcgacggcgcggacatgggcccgcgctattggtacgataatcttcgtagtcaggtccgctttgatgaggccgtgtccgcggcagttgcagatggccacgctacatttgttgagatgtctccacatcctgtgctcactgcggcggttcaggaaattgcggcagacgcggtagctattggtagccttcatcgcgatacagctgaagaacatctgattgcagaactggcgcgcgcccatgtccatggcgtggccgtggactggcgtaacgtgttccccgcggccccgcccgttgcgctgccgaactacccattcgagccgcaacgctactggcttgcccctgaagttagtgaccagcttgcggattcccgctaccgtgtggactggcgtcctttagccacgaccccggtggatttggaaggcggattccttgtacatggctccgccccggaatcgttgacctcggcagtcgagaaagccggcggtcgtgtggtccccgtggcatcagcagatcgcgaagccttagccgcagcccttcgtgaggttccaggtgaagtggccggggtgctgagtgtgcacaccggtgcggcgacccacttagccttgcatcaatccttgggagaggctggtgttcgtgcgccgctgtagagacccta

SEQ ID NO: 6 - DNA, 1145 bp, Artificial Sequence
  DNA fragment
tagggtctcactgtggcttgtcacatctcgtgccgtcgctttgggtgaaagtgagccggtggatccggaacaggcaatggtttggggccttggccgtgtgatgggcttagaaacaccggagcgctggggcggcttggttgaccttccggcggagcctgctccaggcgatggggaagcttttgttgcctgcctcggggccgacgggcacgaagatcaggtggctattcgtgatcacgcacgctacggccgtcgtttagtgcgtgcgccgctgggaacacgtgagtcgtcgtgggagccggccggcacggcgctggttacgggtggcaccggggcgctgggcggtcatgtcgcacgccacctggcacgctgtggagtggaagatttagtgttggtcagccgtcgtggcgttgacgcaccgggcgctgcagaactggaagcggagctggtggccctgggagcgaaaacgacaattacagcttgtgacgtcgcagaccgcgagcaattgtcgaagttgctggaagagcttcgtggtcaaggccgtcccgtgcgcactgttgtacatacagcgggcgtgcccgagtcccgtccgctgcacgagattggtgagctcgaaagtgtatgcgcggccaaagtaaccggcgcgcgcttgcttgatgaactctgcccggacgccgaaacctttgttctgttctcgtcgggagctggggtgtggggctcggctaatctgggcgcgtactccgcggcgaacgcttatttagatgcgttggcgcaccgtcgccgtgcggaaggtcgcgcggcaacgtcggtggcctggggtgcgtgggcaggcgaaggtatggccaccggtgatttagaaggcctcactcgccgtggcttgcgcccgatggctcccgagcgcgcgatccgcgccctgcatcaagcactggataatggggatacctgtgttagtatcgcggatgttgactgggaacgcttcgcagtcggcttcacggcagctcgtccgcgtccgctcctcgatgaattagtgactcccgccgtgggagccgttccggccgttcaagcagcgcctgcacgtgaaatgactagccaagagcttttagagtttacgcatagccatgtggctgccattttgggaagagacccta

SEQ ID NO: 7 - DNA, 1157 bp, Artificial Sequence
  DNA fragment
tagggtctcagggacatagttctcccgatgcagtcgggcaagatcaaccgtttaccgaattaggctttgactcgttgacagcagtggggcttcgcaaccaactccagcaggcaacgggcttggcccttccagcaacccttgtctttgagcacccgacggtgcgtcgcttagccgaccacattggtcagcagttggactctggtacgcctgcgcgtgaagcatcgagcgctctgcgtgatggctaccgccaagccggggtttccggtcgtgtacgctcgtacctggacttattggcgggcttgagcgactttcgtgagcacttcgacggttcggacgggtttagccttgacctggtcgacatggcggacggacccggtgaagttaccgtaatctgttgcgcgggaacagctgcgatttcaggccctcacgagtttacgcgtttggccggtgctttacgcggaatcgccccagtacgcgccgttccgcagccgggttatgaggaaggggaaccgcttccgtcgtccatggcagcagtggcagcagtgcaggccgatgcagtgatccgcacccaaggcgataaaccttttgttgtagcgggccattctgccggcgccttaatggcgtatgcccttgcgacagaactcttagatcgcggccacccgccgcgtggagtagtcttgattgacgtctacccgccagggcatcaagacgccatgaacgcgtggttagaggaactcaccgcgacgttatttgaccgtgaaacggtgcgtatggatgatacgcgcttgaccgcacttggcgcctatgatcgcctgaccggccaatggcgtccgcgtgagacaggtttgcctactttgcttgtgtcggccggcgagcccatgggtccctggcccgacgattcgtggaaaccgacctggccgttcgaacatgacaccgtggccgtgcctggggaccattttaccatggtgcaggaacacgcagatgctatcgcccgccacattgatgcgtggcttggcggtggtaatagctagtagcataaccccttggggcctctaaacgggtcttgaggggttttttgcgcgacttccagagaagatgactactgacttgagcgttccaaaacttagcaggtggtcttgggccaaaatgagacccta

SEQ ID NO: 8 - DNA, 1150 bp, Artificial Sequence
  DNA fragment
tagggtctcatcgtccagccgttgctggtggccgccccgccgaacttcctacatatccatttgaacatcaacgcttttggccgcgcccgcatcgccctgcggacgtgagcgcattgggtgtacgcggggccgagcatccgttgctgctggctgcggtagatgtcccaggccatggcggtgcggtgttcacgggccgtctgagtacagacgagcaaccgtggctcgctgagcatgtggtaggcggccgcaccttagttccgggttctgtgctggttgacctggcactcgcagcgggtgaagatgtaggtttacctgtgttggaagagttggtgcttcagcgcccgttagtgttagcaggggccggggcgcttctccgcatgtcggtgggagcccccgacgaaagcggacgtcgcacaatcgacgttcatgcggcggaagatgtagcggacttagctgatgcgcaatggtcacaacacgcaacgggcacgctggcccaaggcgtggccgcgggtccgcgtgacaccgaacagtggcccccggaagatgcggtgcgcatcccgcttgacgatcactatgacggactcgcggaacagggctatgaatacggaccttcgttccaagccttacgcgcggcgtggcgcaaggatgatagtgtctatgcagaggtttcgattgcggcagacgaagaaggttatgccttccatccggtccttttggatgcggttgcccaaaccttgtcgttaggggctttaggcgagccgggtggcggcaaattgccgtttgcatggaacactgtgacactccacgcgtccggggctactagtgttcgtgtggtggcgacgccagcgggcgcggacgcaatggcgctccgcgtgacagaccccgcagggcatctggtcgcgacggtcgattcattggtggtgcgcagcaccggtgagaaatgggaacagcccgagccgcgtggcggtgagggcgaattacatgcactggactgggtgcgtctcgcggaaccggggtcgaccggacgcgttgttgcagcggacgccagtgatttagacgcagtccttcgcagtggagagccggagccggatgccgtgctggtacgctacgaaccagagggtgatgacccgcgcgcagccgagagacccta

SEQ ID NO: 9 - DNA, 1133 bp, Artificial Sequence
  DNA fragment
tagggtctcagaacgcgagcatcgtgaaaccactgcccacgatggtcgcccagtgccgttagtggtgagcgcgcgtagcacggcggcacttcgcgcccaagcggcacaaattgccgaactcttagaacgcccggacgcagatcttgctggcgttggattaggcctggccactacccgtgcgcgccatgaacaccgcgcggctgtcgtggcgtccacacgtgaagaagcggttcgcggtctgcgcgaaatcgcagccggtgcggccactgcggatgccgtagtggaaggcgttaccgaggtggacggtcgcaatgtggttttcctctttcctggtcagggctcgcagtgggcgggcatgggcgcagaactcctttcaagcagtcctgttttcgcaggaaagattcgtgcgtgcgacgaaagcatggcgccgatgcaagattggaaggtttctgatgtgttacgccaagcaccaggagcgccaggcctcgaccgcgtagacgtagttcaacccgtgctgtttgctgtcatggtgtcgttagctgagctttggcgctcatacggcgtggagccggcggctgtcgtgggccattctcaaggtgaaattgcagcggcccacgtggcaggagcactgaccttggaagatgcggcaaaactcgtcgtgggtcgcagccgcctgatgcgctcattgtccggagagggcggcatggcggcggtggcgcttggtgaagcggcggtgcgtgagcgtctccgtccgtggcaagatcgcctgtcagtagctgcagttaatggccctcgcagcgttgtagtaagtggcgagccgggtgcgcttcgcgccttttcagaggactgtgcggccgagggcatccgcgtccgtgacatcgacgtcgattatgccagccattcacctcagatcgagcgcgtccgtgaagagctgctggaaaccactggagacattgccccgcgccccgcgcgcgtgacgtttcattcaactgtggaatcccgctcgatggacggcaccgaactggatgcccgctactggtaccgcaatctgcgtgagacggtgcgctttgcggacgcggtgactcgtttggccgagagcggttatgatgcgtttatcgaggttagagacccta

SEQ ID NO: 10 - DNA, 1134 bp, Artificial Sequence
  DNA fragment
tagggtctcatcttatgttgataagggcggtttcctggatgacgccgcaggatttgacgccgagttcttcggcgttagcccgcgtgaagccgccgccatggatccccaacaacgtttacttctcgaaacgagctgggaattagtggagaacgcgggtattgaccctcatagtctgcgcggaaccgcgacgggtgtgtttctgggcgtggcgaagttcgggtacggagaagatacagccgcggctgaagatgttgaaggctacagcgtgactggcgtcgcacccgcggttgcctctggtcgtattagctatacgatgggcctggaagggccgagcatcagcgtggacactgcgtgcagcagctcgctggtggcgttgcacctggccgttgagagtctgcgcaaaggtgagagtagtatggcggtagtgggtggtgccgccgtcatggcgacgcccggagtctttgtcgacttctcccgtcagcgcgcactcgccgcagatggacgtagtaaagcgtttggcgccggtgccgatggtttcgggttctcagagggtgtcactcttgtgttactggagcgtctttcagaggcacgtcgtaatggacacgaagttttagctgttgtgcgtggatcggcgttaaaccaggatggcgcatccaacggattgagcgcgccatcgggcccggcccaacgccgcgtaattcgccaagcgttagaatcgtgtggtcttgaacctggcgatgttgatgcggttgaggcccacggcaccggcactgctttaggcgacccgatcgaagcgaacgccctgctggacacctatggacgcgatcgcgatgcagatcgcccgctttggttaggctcagtcaagagtaatattggacacacccaggcagcagcgggtgttaccggcttacttaaggtggtcctggcattacgtaacggcgagctgccagccaccttacatgttgaggagcccacaccgcacgtcgattggtcatctggcggtgtggccctgttagccgggaaccagccgtggcgccgcggggagcgtacccgtcgtgcggcagtgtcagcatttggcatctcgggtaccaatgcccatgttatcgtagaagaggccccggaacagagacccta

SEQ ID NO: 11 - DNA, 1173 bp, Artificial Sequence
  DNA fragment
tagggtctcaaaattcttcgcgaagtggtgggcctgcttggcgctggagaactggatcgtctgccggtttcagcctgggaattaggcagcgcacccgcagcgcttcagcacatgagccgcggacgccacgtcggcaaactggtcttgacccaaccggctccggtagatccagacggcactgtgctgattactggcggaacaggaactctgggtcgcttactggcccgccacttggtcacggaacacggcgtgcgtcatctgcttctggtttcacgtcgcggcgcagacgcccctgggagtgatgaacttcgcgcagaaatcgaggacttaggtgcgagcgcagaaatcgcagcgtgcgatactgcagatcgcgacgccctgtcggcgcttcttgatggcctgcctcgtcccttaaccggagtcgtgcatgcagccggtgtcctggccgatggcctggtcacaagcatcgatgaaccggcggtcgagcaagtacttcgcgcaaaagtggatgcggcatggaatctgcacgagttaaccgccaatacgggcctctccttctttgttctgttcagttccgcggcgtcggttctcgcgggaccgggacagggtgtatatgcagccgctaacgaaagcctgaatgccctggccgcgcttcgccgcacacgtgggttaccggccaaagcgctcggatggggcttgtgggcacaggcgtcggagatgacgtccggccttggcgaccgcatcgcgcgtactggtgtagcggcgctgccaacggaacgcgccctggccttgtttgatagcgcgttacgtcgcggcggtgaagtagttttccctctgtcaattaaccgcagcgcattgcgtcgcgcggaattcgtgccggaagtgctgcgtggtatggtccgcgcgaagttgcgcgcggcgggccaagccgaagcggcgggcccgaacgtcgtggatcgcctcgccggccgttccgaatcagaccaggtcgcgggtcttgcggagcttgtgcgttcacatgcagcggctgtctccggctatggcagcgcggatcaattaccggagcgtaaagcatttaaggaccttggctttgacagccttgcggccgtagagctgcgcaatcgtctgggcactgcgaccggtgtacgtttgccttcaacgctagagacccta

SEQ ID NO: 12 - DNA, 1150 bp, Artificial Sequence
  DNA fragment
tagggtctcagccgctcgccacggcgtattatgggcagccgcgttggtccgccgctggcttgaacaggaagagttaccgggcgccactctggttatcgcgactagcggcgcggtcacagtctctgatgacgactcggtgccggagccgggcgcggcggccatgtggggcgtgatccgttgtgcacaagcggagtcaccggatcgctttgttctgctcgatacagatgccgagcccggaatgctgccggcggtgccggacaatccccaactggcgttgcgtggtgacgatgtatttgtgccgcgtttatccccgctcgcaccttcggcactgactttaccggcgggtacccagcgtcttgtacccggagatggggccattgattccgtagccttcgagccggcgcctgacgttgagcaaccgctccgtgccggcgaagtgcgtgtagatgtccgcgcgaccggtgttaacttccgcgacgttcttcttgcactgggcatgtacccgcagaaggcagatatgggaacagaggccgcgggcgtagtaacggcagttggcccggacgtggacgctttcgcccccggcgatcgtgtactgggacttttccaaggcgcctttgcgccgattgcggtaacggaccatcgcctgttggcacgtgttccagacggatggagcgacgcagacgctgctgcggtacctattgcgtacaccacagcgcattacgccctgcacgatttagccggccttcgtgcaggccagtcagtgcttatccatgccgcggccggtggcgttggtatggctgccgtggcccttgcgcgccgtgccggcgcggaagttttagccacagcgggtccagccaaacatggcacgttacgtgcgctgggcttagacgatgaacacattgcgagttctcgcgagacaggttttgcgcgtaaattccgtgagcgtaccggtggacgcggcgtcgatgtagtgttgaacagtttaaccggcgaactcttagacgagagcgccgaccttcttgcagaggacggtgtattcgtagaaatgggtaaaaccgatctgcgcgacgcaggcgatttccgcggccgttacgcgccgtttgacttgggcgaggcgggcgatgaccgcctcggcgaaatagagacccta

SEQ ID NO: 13 - DNA, 1141 bp, Artificial Sequence
  DNA fragment
tagggtctcattgaccaattttggtagcatctcagaggtggcgccggaagaatttgcggaaaccattgcggcgaaaaccgccctcttagccgtactggatgaagtccttggtgaccgtgcagtcgagcgtgaagtgtactgttcgtctgtggcgggtatttggggcggtgcgggtatggcggcgtacgcggcgggtagtgcgtacctcgacgcattagctgagcatcaccgtgctcgtggtcgtagctgcacgtcagtggcatggacgccgtgggcattacccggcggcgcggtggacgacggttatctccgtgagcgcggcctgcgcagcttgagcgctgatcgcgcgatgcgtacctgggagcgtgtcttggcagcgggtcccgttagcgtggcggtcgccgacgtcgattggccggtactgagcgaaggattcgcagcgacgcgcccgaccgccttattcgccgaattagccggccgcggcggacaagctgaagccgagcccgatagtggccccactggcgagccggcgcagcgcttggcgggcctctcacctgacgagcagcaggagaacttacttgagttagtcgcaaatgccgtggcagaggttttaggccatgagtcggcagccgaaatcaatgttcgtcgcgcgttctctgagcttggattggattctctgaatgctatggctcttcgtaaacgtttatctgccagcaccggattacgccttcctgcgagcttggttttcgaccacccgacagttactgccctggcgcagcacttacgcgcccgtcttgtcggtgacgcggatcaagctgcggtacgcgtagttggtgcagcggacgaatccgaaccgatcgctattgttggtatcggttgtcgttttccgggcggcattggatcgcccgagcaattatggcgcgttcttgctgagggtgcgaatctgacaaccggtttcccggctgaccgcgggtgggatatcggccgtttatatcatcctgatccggataatccgggcacatcctacgttgataagggcggcttccttacggatgccgcagattttgacccggggttcttcggtattacccctcgcgaggcgctggccatggatccgcagcagcgccttatagagacccta

SEQ ID NO: 14 - DNA, 1168 bp, Artificial Sequence
  DNA fragment
tagggtctcaggtttctccgcacccggtggttgtgcaggccgtggaagaggctgtggaagaggcggatggggcggaagatgccgtggttgttggatctctgcatcgtgacggtggcgatctgagcgcgttcttacgtagcatggccaccgcccacgtttcaggggtcgacatccgttgggacgtagcattgccgggtgctgcgccgttcgcactgccgacgtacccgttccaacgcaaacgctattggcttcagcctgcggcaccggcggccgccagcgatgagcttgcgtaccgtgtgagctggacccctattgaaaagccggaatctggcaacctggacggcgattggctcgttgttacgccgctgattagcccagagtggacagaaatgttatgtgaagccatcaatgccaatggcggccgcgccttacgctgtgaggtggacaccagcgcgtcccgtactgaaatggctcaagccgtggcccaggccggtaccggcttccgtggagttctgtcattattaagcagtgatgagagcgcctgtcgtccgggcgtgccggcgggcgccgtagggcttctcactttggtccaagccctcggcgacgcaggcgtcgatgcgcccgtttggtgtctgacccaaggagccgttcgtaccccggcagatgacgatctggcccgcccggcccagacaaccgcacatggattcgcccaagttgccggcctcgaattaccgggccgttggggtggcgtcgttgatcttccggagagcgtggacgatgcggcactgcgtttattagtggctgtgttgcgcggtggcggccgcgcagaggaccacctggccgtacgtgatggccgtttgcatggccgccgcgtcgtacgtgctagcctgccgcagagcgggtcacgttcttggactccccacggcactgtattggtcactggggctgcttcgcccgtcggtgaccaactcgtgcgttggctcgccgaccgtggcgctgaacgtttagtccttgcaggcgcgtgcccgggagacgatctgctggccgccgtggaagaagctggcgcctcagcagtagtgtgtgcccaagacgccgcggccctgcgcgaagcgctcggcgatgaacccgttaccgcccttgtacacgcgggtaccttgaagagacccta

SEQ ID NO: 15 - DNA, 1152 bp, Artificial Sequence
  DNA fragment
tagggtctcatgatgcggcctggacgctggccacgggtcgtgcccgttttgacgtacgcgccgcggttttaggcgacgaccgtgcgggtgtgtgtgccgagttagatgccttagcggaagggcgtccctcagcggatgccgtagcgccggtcacttccgccccgcgcaaacctgtactcgtctttccgggtcagggtgcgcaatgggtcggtatggcccgtgatctgctggagagtagcgaagttttcgcggagtccatgagccgttgcgcagaggccctgtcaccccataccgattggaagctcttggatgttgttcgcggtgatggcggaccggatcctcacgagcgtgtcgatgtgttacagccggtgctgttcagcatcatggtttctcttgcagagctgtggcgcgcgcacggcgtaaccccggcagcggtcgtaggtcactcacaaggcgaaatcgctgcggctcatgtagcgggcgcgcttagtcttgaggccgcagccaaagtggtggcgctccgctcccaggtattgcgtgaactggacgatcagggtggcatggtgtcggtgggcgcaagccgtgacgaactggaaaccgtgcttgcgcgttgggatgggcgtgtcgccgtggcagcggtcaacgggccgggtacctcggtggtcgccgggccaacggccgaattggatgagttcttcgccgaagccgaggctcgcgaaatgaagccccgtcgtatcgccgtacgctacgccagtcattcgccagaggtagcccgtattgaggaccgtcttgcagcagagctgggtacaatcaccgcggtccgtggttcagtgccgctgcatagcactgtaaccggggaagtaatcgatacctcagcgatggacgcgtcctattggtatcgtaacttacgccgcccggttttattcgagcaagcagttcgtggactcgttgagcagggcttcgacaccttcgtcgaggtcagtcctcatcccgtgctcttgatggctgtagaagaaaccgcggagcacgcgggtgccgaggtaacttgtgtacccacattacgtcgtgagcaaagcggccctcatgagttcttacgtaacttattacgtgcgcacgtgcacggagttggcgccgatcttcgtagagacccta

SEQ ID NO: 16 - DNA, 1159 bp, Artificial Sequence
  DNA fragment
tagggtctcattatgcttgagacggcctgggaagccgtagagcgtgcaggcatcgaccccgacgccttacgcggaacggacacaggagttttcgtgggcatgaacggacaatcttatatgcaattacttgcgggtgaggcggaacgcgtcgacggctaccagggcttgggtaacagcgcgagcgtcctcagcggccgcattgcctacacgttcggttgggaaggtcctgcgttaacagtggatactgcatgttctagcagtttggtgggtattcatttagcgatgcaagcccttcgtcgcggcgaatgctcactcgctttggcgggtggcgtaacggtcatgtctgacccgtacaccttcgttgatttcagcacgcagcgtggccttgcgagtgacggtcgctgtaaggccttcagtgcgcgtgcagacggtttcgccttatcagagggtgtcgcggccttagtgttggagcccctcagtcgtgcgcgtgctaatggccaccaagtgcttgccgtcttgcgcggcagcgcggtcaatcaggacggtgccagcaacgggctggcggcccctaatggtccgagccaggaacgtgtgattcgccaagccttagccgcgagcggagtgccggcggcagatgtggacgtggtagaggcccacggtacaggcacagaactgggtgacccgattgaggccggagcgttgattgccacgtatgggcaggaccgcgatcgtccactgcgtctgggaagcgtgaaaaccaatattggccatacgcaagccgctgcaggggcggctggtgtcatcaaagtcgtgctcgcaatgcgccacggtatgttgccacgctcgcttcacgcagatgagttaagccctcatattgactgggaatctggcgccgtggaagtgctccgtgaggaagttccgtggccggccggggagcgtccacgccgcgcaggcgttagctcgtttggcgttagcggaactaatgcccatgtgattgttgaagaagccccggcggaacaagaggccgcccgcaccgaacgcggtccgctgccgtttgtgctctcgggccgctccgaggcggttgtcgcggcgcaggcacgtgccttagccgaacatctgcgtgatacacctgagttaggcctgactgatagagacccta

SEQ ID NO: 17 - DNA, 1131 bp, Artificial Sequence
  DNA fragment
tagggtctcaagaagatggctggacggtggaagtacgctcggcattagccgaggcaggagcggaaccagaggttacgcgtggagtgggtgggctggttggtgattgcgcaggggtcgtcagcctgctggccctcgaaggggacggcgccgttcaaacgctcgtactggtgcgcgaattagatgcggaaggcattgatgcgccactctggacggttactttcggtgcagttgatgcggggagcccggtcgcacgtcctgaccaggccaaactctggggtctgggccaagtggcgtcattagaacgtggcccgcgctggactggtctggttgacctgccgcacatgccagaccctgagcttcgtggacgcctgacggccgtccttgccggaagcgaggaccaagttgcggttcgcgctgacgccgtgcgtgcccgccgtctgtcaccggctcacgttacagcaacgtcagaatatgctgtcccgggcggcacgatcttagtgacaggcggcacggcaggattaggtgccgaggttgctcgctggttagctggccgcggggccgaacatttggcactggttagccgccgcgggcctgataccgaaggcgtaggtgacttaaccgccgagctgacacgcctgggtgcgcgcgtgagtgtgcatgcatgtgatgttagctcacgtgagccggtgcgcgagcttgttcatggcctgattgaacaaggcgatgtagttcgcggagttgtgcatgcagcaggtttaccccaacaagtggccatcaatgacatggatgaggcagcgtttgacgaagtagttgcagcgaaagcgggcggggccgtgcacctggacgaattatgctcagatgcggaactgtttctcttatttagctccggtgccggtgtatggggctctgcccgccagggagcgtatgcggcgggcaacgcctttctggacgcgttcgctcgccaccgccgtggtcgtggtttacccgcgactagcgtggcgtggggactctgggcggcgggcgggatgaccggcgacgaggaagccgtctcattcttgcgtgaacgtggagtccgtgcgatgccggtaccgcgcgccctggcggcgctcgaccgtgttctgagagacccta

SEQ ID NO: 18 - DNA, 1167 bp, Artificial Sequence
  DNA fragment
tagggtctcaatgggaaggcatggcccgcgagctcctgccagtaccggtgttcgcagaaagtattgcggaatgcgatgctgtgctgagcgaagtggccggattttccgtctctgaagtactggagcctcgtccggatgcgccgtctctggagcgtgttgacgtagtgcaacctgtgcttttcgccgtgatggtgtcactggcccgcctgtggcgcgcatgtggcgcagtcccatctgccgtgattggccattcacagggcgagattgctgcagcagttgtagctggtgcgttgtccttagaggacggcatgcgcgttgttgcgcgccgctcgcgtgccgtccgcgctgtagcggggcgcggctccatgctgtcggtccgtggtgggcgctcagacgttgagaaactgttagccgatgacagctggaccggccgcctggaagtagccgccgtcaacggtcctgatgcagtggtcgtggccggcgacgcgcaggcagcgcgcgaatttctggagtactgcgaaggcgtaggcattcgcgcccgtgcaatcccggtggactatgcatcgcacacggctcatgtggaaccggttcgtgatgagttagtacaagccctcgcggggattacacctcgtcgcgcagaagtacctttcttctcgaccttgactggtgacttcctggacggcacggagcttgacgccggctactggtatcgcaatctgcgccatccggtcgaatttcactctgcagtccaagctttaacggatcaagggtacgcgacctttattgaggtgagtccgcatcctgtgctcgcatcaagcgtgcaggaaacccttgatgatgcagaatccgacgccgcagtacttggaaccctggagcgcgacgctggtgatgcggatcgctttctgactgcacttgcggatgcgcacacgcgcggagtcgcagtcgactgggaagcggtactgggacgcgcagggttggtggatcttcctggataccctttccaaggtaaacgcttctggctgctgccggatcgtacgactccgcgcgatgaattggatgggtggttctaccgcgtagattggacagaagttccgcgtagcgaacccgccgcgctgcgcggccgttggcttgtggttgtgccggaaggacacgaagaaagagacccta

SEQ ID NO: 19 - DNA, 1133 bp, Artificial Sequence
  DNA fragment
tagggtctcatgtagttcgtctctggtggctctgcacaccgcatgcggcagcttacgcgacggcgactgtggcttggcagttgcaggcggtgtgtcagtgatggccgggcctgaagttttcaccgaattttcgcgtcaaggtgccctttctcctgacggacgctgcaaaccctttagcgatgaggccgacggctttggtcttggtgaaggtagcgctttcgtcgtcctgcaacgtcttagtgatgcacgccgtgaaggccgccgcgtgttaggcgtggtggcgggcagtgctgtgaatcaggacggtgcatcgaacggattaagcgcgcccagcggagtggcgcagcaacgcgtcattcgtcgcgcatgggctcgtgcaggtattacaggtgcagatgtcgcggtggtcgaggcgcacggtacaggcacccgccttggtgaccctgtggaagcctcagcccttttggccacgtacggtaaaagccgtggctcgtctggcccggttttactcggatctgtgaaaagcaacattggacatgctcaggccgcagccggcgttgctggtgtgattaaagtcctgcttgggcttgagcgtggagtagtgccgcccatgctgtgccgtggcgagcgttccggtctgattgattggtctagcggtgagattgaacttgccgacggtgtccgcgagtggtcccctgcagccgacggggttcgtcgcgcgggagtaagtgcattcggtgtaagtggtaccaacgctcacgtgattattgcagaaccgccagaacccgagccggtcccgcaacctcgtcgcatgttaccggcgactggcgtcgtgcctgtcgtgctgtctgcccgtacaggggcggcactgcgcgcccaagctggacgcttagctgatcacttagccgcgcacccgggcattgctccagccgacgtcagctggaccatggctcgtgcacgccaacacttcgaagaacgcgccgccgtattggccgcggacaccgcagaggccgtgcatcgtttgcgcgccgttgccgacggagcagtcgttcctggcgtggtcacaggtagcgcctctgacggtggttcggttttcgttttccccggccagggcgcccaatggagagacccta

SEQ ID NO: 20 - DNA, 1184 bp, Artificial Sequence
  DNA fragment
tagggtctcaactctggatcatggccagacgagcgtaagtgtggtggacatggatcgccgccgcttcgttgaactctttacagcggcccgtcatcgtccgcttttcgatgaaatcgccggagcacgcgcggaagcccgtcagtcagaagaaggtcctgccctcgcacagcgtttagcggcactgagcacagcggagcgccgcgagcacttggcgcacctgatccgcgctgaggtggccgctgtgctgggacatggggatgacgcggcaattgatcgcgatcgtgctttccgtgacctcggctttgacagcatgaccgcggtggacttacgcaatcgccttgcggccgtcacgggtgttcgcgaggcggcgaccgtggtatttgatcacccgacgatcactcgcctcgcagaccactatcttgaacgcctggtcggcgcagccgaggcggagcaggcgcctgcgttggtgcgcgaagttcccaaagatgccgatgacccgattgcaattgtgggaatggcctgccgctttccgggcggtgtgcataatccgggtgaactgtgggagtttatcgtgggcggcggcgacgccgtcactgaaatgcctaccgatcgtggctgggacttagacgcgttattcgatccagatccgcagcgccacggtaccagctattcccgtcacggcgcattcttagatggcgcagccgactttgacgcggcgttctttggtatctccccgcgcgaagcgctggccatggatccacaacaacgccaggtgctggagacaacatgggaactgttcgaaaatgcaggaattgatccgcatagtctgcgcggtagtgataccggcgtgtttcttggtgccgcctaccagggatacggtcaagacgcggttgtccccgaggacagcgaaggttatctgctcactggtaattcatcggccgtcgtttcgggtcgcgtggcgtatgttctcggtttagagggccctgccgtaaccgtagacactgcctgttcgtcgagtttggttgccctgcactcggcatgcggttctttacgtgatggtgattgtggcctcgctgtagctggtggcgttagcgtaatggcggggcccgaggtattcacggaatttagccgtcagggtgggctggcggtggacggacgttgtaaggctttctcaagagacccta

SEQ ID NO: 21 - DNA, 1165 bp, Artificial Sequence
  DNA fragment
tagggtctcacgaactgtcggatgcgatccgctctgggctcgaacagtcaggagcgaccgtgttaacctgtgacgtggaaagccgtagtacgattggtaccgctcttgaagccgcggatacagatgccctgagcaccgtagtaagcctgctttcgcgcgatggcgaagccgtggatccatcgctggacgcgttagctctcgtgcaagcgttgggcgctgcgggagtagaggccccgttatgggtgttgacccgtaacgcggtgcaggttgcggatggggaattagtggacccggcgcaagcaatggttggcggtcttggtcgcgttgttggaatcgaacaacctggccgctggggtggtttagtagacttagtcgacgcggatgccgcaagcattcgtagccttgcggcagtactggcggaccctcgtggtgaagagcaagtcgctattcgtgcagacggtattaaagttgcccgtctggtgccggcccctgcccgcgccgcacgtacgcgctggagccctcgcggaaccgtgttagtaaccggtggcaccggtggtatcggcgcccacgtggcgcgctggttagcgcgttcgggtgccgagcatttagtgctgttgggccgccgcggcgctgatgcccctggggcttcagaactgcgtgaagaacttactgccttggggaccggtgttaccatcgcagcctgcgatgtcgcggatcgcgcgcgcttagaagctgttttagccgcggaacgtgcggaaggccgtactgtgagtgcggtcatgcatgccgcaggcgtttctacgtctacaccccttgatgacctcaccgaggcggaattcaccgagatcgccgatgtgaaggtccgcggcactgtgaacctggatgaactttgcccggacctggacgcgtttgtgttattctccagcaacgcgggcgtatggggctctccgggcctggcgagctacgcggctgcgaacgctttcctggacggttttgcccgtcgtcgtcgttcggaaggggcccctgtgacttcgattgcatggggcctgtgggcgggacagaatatggcgggcgacgagggcggagagtacttacgtagccagggcctgcgcgctatggacccggaccgcgcagtagaagaattacatattactcagagacccta

SEQ ID NO: 22 - DNA, 1129 bp, Artificial Sequence
  DNA fragment
tagggtctcaaggtgtttgccgattcaattcgtgactgcgagcgtgctttagctccacatgtcgactggtcattaacggacttgctctctggcgcccgcccgctggatcgcgtggacgtggtgcagcctgcgctctttgcagtgatggtgtcattagcggccttatggcgttctcacggggtcgagcctgccgccgttgtaggccattcgcaaggtgagattgcggctgcccacgtagcgggtgcacttacgttggaagatgctgctaaacttgttgcagttcgttcgcgtgtgttacgtcgtttaggcggccagggcgggatggcaagcttcggcctcggtaccgaacaagcggccgagcgtatcggccgctttgcgggtgccttatctattgcctcggttaatggaccgcgttcggtggtggtagccggagagagcggcccgctggacgaattaatcgccgagtgtgaggctgagggcattaccgcgcgtcgtatcccggtggattacgcctcgcattcaccgcaggtagagagcctgcgcgaagagctcttaacggagttagccggtatttcaccggtttccgctgacgtagccttatattcaacgaccacaggccagcctattgatacagcaacaatggacaccgcctattggtacgcgaacttacgcgagcaagtgcgcttccaagatgcgacccgccaattagcagaggcaggctttgacgctttcgttgaggtaagtccgcacccggttttgaccgtgggaattgaggccaccttagacagcgcactgccggcagacgcgggtgcatgtgtcgtgggcactctgcgccgcgaccgcggcggtttagccgattttcacacagccctgggcgaagcctatgcccagggtgtagaagttgattggtcgcctgcgtttgcagacgcgcgccctgtggaactgccggtttaccctttccagcgccaacgttattggcttccgattccaactggtggccgcgcgcgcgatgaggacgatgactggcgctaccaggtggtttggcgcgaggccgaatgggaatcagcatctctggcgggtcgcgttctgttagtaaccggtccgggtgtcccgtccgaaagagacccta

SEQ ID NO: 23 - DNA, 1165 bp, Artificial Sequence
  DNA fragment
tagggtctcagatacagcctgcagcagtggcttaactgctctgcaccttgcaatggagagtttacgccgcgatgaatgtggtcttgcgttagcaggcggtgttactgttatgtctagtccaggcgcgttcacggaatttcgttcgcagggtggactcgcggccgacggccgttgcaaaccattttcgaaagccgcggatggtttcggcttagccgaaggcgcgggtgtccttgtactgcagcgtctgagcgctgcgcgtcgcgagggtcgcccggtattggcagtcctgcgcggtagcgcggtaaaccaagatggagcatcgaatggtcttacggcgccgtcaggcccggcccagcagcgtgttatccgtcgtgctctggaaaatgcgggcgtccgcgcaggcgatgtggattatgtcgaagctcacggaacgggcacgcgcttaggcgaccccatcgaggttcacgcgctcttatctacttatggcgccgagcgcgatccggatgacccgctttggatcggctccgtgaagagcaacatcggtcacacccaggcggctgcgggtgtggccggtgttatgaaggcagtgttagcgctgcgccatggcgagatgcctcgcacgctgcatttcgacgaaccgtcaccgcagatcgagtgggacttaggtgccgtttctgtggtgtcacaagcgcgcagctggccagcgggcgagcgcccgcgccgcgcaggagtgtcatcttttggtatctctggcactaacgcacacgtcatcgtggaagaggcgccggaagcagatgagccggaacccgctccggacagtggcccagttccacttgtgctcagcgggcgcgacgagcaagcaatgcgtgctcaagcgggccgtctggcggaccacctggcgcgtgaaccacgcaactcgctgcgtgatacgggatttacattagcaacccgccgcagcgcgtgggagcatcgcgcagtcgttgtgggagatcgcgacgatgccctggcgggtttgcgcgctgttgctgatggccgtatcgccgatcgcaccgcgaccggtcaggctcgcacccgtcgcggcgttgccatggtgtttccgggtcaaggtgcgcagtggcaagggatggcgcgcgacctgcttcgtgagagccaggtagagacccta

SEQ ID NO: 24 - DNA, 1160 bp, Artificial Sequence
  DNA fragment
tagggtctcatagcccagcaacgccgttcagacggcttgccggcgacggcagtggcctggggcacctgggccggctccgggatggccgaaggtccggttgcggatcgcttccgccgtcacggcgtaattgaaatgcccccggaaaccgcgtgtcgcgctctgcaaaacgcactcgaccgtgccgaggtatgtccgatcgtaatcgatgtgcgttgggaccgtttcttactggcctataccgcacaacgcccgacgcgcctgttcgacgagatcgatgatgcgcgccgcgcggccccgcaggcggcggccgagcctcgtgttggagctttggccagtctgcctgcaccggagcgcgagaaagccctgttcgaactcgtgcgcagccatgctgcggcagtactgggccacgcgagcgccgagcgtgtccctgcggaccaagcattcgccgaacttggcgtggactcgttatcggcgcttgaactgcgtaatcgccttggcgcggccaccggcgtacgtctgccgacgacgaccgtgtttgaccatccggatgttcgcaccctggcggcccatctggcggccgaacttggtggtgccactggagccgaacaggcggcgccggccaccaccgcgccggtagatgagccgatcgcaattgttggcatggcgtgtcgccttccgggtgaagtcgactcgccggagcgtctttgggagttaatcacaagtgggcgtgattccgctgccgaagtacccgatgatcgcggctgggtgccagatgagctgatggcctctgacgcagcaggtacccgccgtgcgcacggtaactttatggcgggcgcaggagactttgatgctgcattctttggaatttctccacgtgaagcattggcaatggacccacaacaacgtcaagccttagagactacctgggaagcacttgaaagtgctggtattccgccagagacgttacgcggctcggacacaggcgtattcgtcggcatgagccatcaggggtacgccacaggccgtccgcgtccagaagatggtgttgatggctatctcttgaccggcaatacagccagcgtggcaagcgggcgcatcgcctatgtgctgggcctcgaaggaccggcgttaactgttgatactgcatgtaagagacccta

SEQ ID NO: 25 - DNA, 1181 bp, Artificial Sequence
  DNA fragment
tagggtctcataaacctgtcgcgcgccgcagcacggaagtggatgaagtttcagcactgcgttatcgtattgaatggcgtcctaccggcgcgggcgaaccggcgcgccttgacggcacctggctggtagctaaatatgccggcacggcggatgagacgtcaacagcggcccgtgaagccctggagagcgcgggcgcccgtgttcgcgagcttgttgttgatgcccgttgtggccgtgacgaactcgccgaacgtctgcgcagtgtcggcgaggtagccggtgtactttcactgttagcggtggacgaagccgaaccggaagaagcgccgctcgcgctggccagtcttgcggatactctgtcactggttcaagccatggtgtcagcggaacttggttgtcctttatggactgttactgagagtgccgtagcgaccggtccctttgagcgcgtacgtaacgcggctcacggcgcactttggggagtgggtcgtgtcattgccttagagaacccggccgtctggggcggcctggttgacgttcccgccggctcggttgcggaacttgctcgccacttagcggcggtggttagtggtggagcgggtgaagatcaactggcgctccgtgcggatggagtgtacggccgccgctgggtgcgcgcggcggcccctgcgaccgatgatgaatggaaaccgaccggaaccgtgcttgtgacaggcggtaccggtggggtaggtggccagattgcacgctggctggcacgtcgtggggcgccgcatctgttactggtatcccgctccggaccggacgcagatggcgctggcgagctggttgcggaattggaagcacttggggcacgcacgaccgtagctgcgtgcgatgtgacggaccgtgaatcggtccgtgagcttctgggcggcatcggtgacgatgtacctctctcggccgttttccatgcggcagcaactctggacgacggtacggtggatactttaaccggcgaacgcatcgaacgtgcgagccgcgccaaagtgctgggtgcccgtaatttgcacgagcttacccgcgagcttgacttaactgcgttcgttttatttagtagcttcgcgagcgcctttggggccccgggcttgggtggatacgcgccgggtaacgcctatctggatggattagcagagacccta

SEQ ID NO: 26 - DNA, 1171 bp, Artificial Sequence
  DNA fragment
tagggtctcacattgcggaaggcatgcgctcggccctggcatggtttgcaccgggtgggagcgaggtgccgttttacgccagtctgaccggtggtgccgtagacacccgtgagctggttgcggattactggcgtcgcagctttcgtctccccgtgcgttttgatgaggccattcgtagtgcacttgaagtgggcccggggacgtttgtagaggcatcaccccaccccgtgcttgccgcagcattacagcagaccctcgacgccgaaggctcgtcagccgcggtagtgccaacgttacaacgcggccaaggtgggatgcgccgtttcctgctcgctgccgcgcaagcgtttacgggcggcgtggcggtggactggaccgcggcgtacgatgacgttggggcggaacctggtagtctgccagagtttgccccagccgaagaagaggacgaaccggcagagagcggtgtggactggaacgcaccgccacacgtgctccgcgaacgtctccttgcggtcgtgaacggtgaaacggcggcattagctggtcgcgaggctgatgcagaggcaaccttccgcgaactcggcttggatagcgtcttagcggcccagttacgtgcgaaggtatcagccgccattggacgtgaggtcaatatcgcactgttatacgaccacccaacccctcgtgctctggctgaagcgctggcggcagggaccgaggttgcccaacgtgagacacgcgcacgtaccaacgaggcggcgcctggcgagccggtggccgtcgttgcgatggcctgtcgccttccgggcggtgtatccacaccggaagagttttgggagttgctctccgagggtcgtgatgccgttgcggggttaccgacagatcgcggctgggacctggactcgctgtttcatccggatccgactcgtagtggaaccgcgcatcagcgtggaggagggtttctgactgaggccacggcgttcgacccggccttcttcggtatgagcccgcgcgaagctcttgctgttgacccgcagcagcgcctgatgcttgagctctcttgggaagtgttggagcgcgcgggcattcccccgacctcacttcaagcttcacctacaggggtatttgttggcctgattccgcaagagtacggcccgcgtttagagagacccta

SEQ ID NO: 27 - DNA, 1136 bp, Artificial Sequence
  DNA fragment
tagggtctcattagcggaaggcggagagggagttgagggctacctgatgaccgggacgacgacgagcgtggcgagtggccgcatcgcgtatacgctgggcttagagggccctgctatcagcgtagacaccgcgtgcagtagttcattggttgccgtacatttggcctgtcagagccttcgtcgcggtgagagctctttagcgatggccggtggggtgaccgtgatgcctacgcctgggatgctcgttgacttttcacgtatgaactctctggcacccgatggtcgttgtaaagcctttagcgcaggagctaacggttttggcatggccgagggtgcggggatgctcttgttagaacgcttatcggatgcgcgtcgtaatggtcatccagtactggcggttctgcgtggcaccgcggtaaattctgacggcgcctcaaacggcttgagtgcacctaatggtcgcgcgcaggtacgtgtgattcagcaagctctggcggaaagtggcttgggtccggccgacattgatgcggtggaagcgcatggaacaggtacgcgcctgggcgatccgattgaagcacgcgctctgtttgaagcctatggccgcgaccgtgaacaaccgttacacctcggcagcgtcaaatccaacctgggccacacccaggcggcggctggcgtcgcgggtgtcattaaaatggtcctcgctatgcgcgccggtacgctgcctcgtacgttacatgcttcggaacgttctaaagagatcgattggtcgtcgggcgcaatttctctgttagacgagccggaaccgtggccggcgggagctcgtccacgtcgtgcgggcgttagctcattcggcatctccggcacgaacgcccacgccatcatcgaagaagcgcctcaagttgtagagggcgaacgcgtcgaagcaggagatgttgttgcaccctgggttctctcagccagcagcgccgagggcttacgtgcgcaggcggcccgtcttgccgcgcatctgcgtgaacacccgggccaggacccacgcgatattgcgtatagtcttgcaactggacgcgcggccctgccacaccgcgccgcatttgcacccgtggatgaaagcgccgccctgcgcgtgagagacccta

SEQ ID NO: 28 - DNA, 1158 bp, Artificial Sequence
  DNA fragment
tagggtctcacgtgcttgatggtctggccacagggaatgccgacggcgcggcagttggtaccagtcgcgcacagcaacgcgccgtgtttgtatttcctggtcagggttggcagtgggctggcatggccgtggatttgctggatacaagccctgtgttcgccgctgcattacgtgagtgtgcggacgcactggaaccgcaccttgactttgaagtaattccgttcctgcgtgccgaggcagcacgtcgtgaacaggatgcggcgttatctactgaacgtgtggatgtcgtgcagccagttatgttcgcggtgatggtatcgttagccagcatgtggcgcgcccacggggttgaaccggccgcagtgattggtcacagccaaggggaaatcgcagcagcttgcgttgccggcgcgttaagtctggacgacgcagcccgtgtggtagccttacgtagccgcgtgatcgccactatgccgggcaacaaagggatggcaagcattgcggcaccagcgggcgaggttcgtgcccgcattggagatcgcgtcgaaatcgcggcggtaaacgggccgcgtagtgtggttgtggccggtgactccgatgagttagatcgcctcgtggcatcctgcaccacggaatgtattcgcgcaaaacgtctcgcagttgactacgcgtcacattccagccatgtcgagactattcgtgacgcgctgcatgcagaattaggtgaagattttcatccgcttcccgggtttgtgccgttcttctccacggtaaccggccgctggacgcagcctgacgaacttgacgccgggtattggtatcgtaacctgcgtcgtaccgtgcgtttcgcggatgccgtacgtgcccttgcagagcaaggatatcgtacgttcttagaagtgagcgcacacccgattctcacagcggcgatcgaagagattggtgatggcagcggagcggacttgagcgcaattcattccttacgtcgtggcgacggctcattagccgattttggcgaggcgctgagccgcgcgtttgccgccggtgtcgccgtggattgggagtccgttcatcttggtaccggggcgcgtcgcgttccactgcctacctatccctttcaacgcgagcgtgtgtggttggaacctaaaagagacccta

SEQ ID NO: 29 - DNA, 1126 bp, Artificial Sequence
  DNA fragment
tagggtctcacgctggtgtttgaccacccgacgcccctcgctgtagcggagcaccttcgcgaccgcctcttcgcagcgagtccggcggttgacattggtgaccgtctcgacgaacttgaaaaggcattagaggctctcagcgcagaagatgggcacgatgatgttggtcaacgcctggagagcctgctccgtcgctggaattcccgccgtgctgatgcaccgagcaccagcgcgatctctgaagatgcatctgacgatgaactgtttagcatgttggaccagcgttttggcggcggcgaagatctctagtagcataaccccttggggcctctaaacgggtcttgaggggttttttgaggacgcgttgcgcagatgtacgacaatatctccgcttctagtacctcactaatacgactcactatagggagaagctgtcaccggatgtgctttccggtctgatgagtccgtgaggacgaaacagcctctacaaataattttgtttaatttgtttaactttaagaaggagaatgagtggagacaatggcatgacggaagagaaactgcgtcgttatctgaaacgtactgtcactgaattggatagtgtgacagcgcgcctgcgtgaagtcgaacaccgcgccggcgaaccgattgcgattgtggggatggcatgccgtttcccaggtgacgtagattcgccggagagtttctgggagtttgtaagcggcggcggtgacgcgattgcggaagcgcctgcggatcgtggctgggagcctgatccggatgcacgtcttggtggaatgctggcggcggcaggggattttgatgccggcttcttcggcattagcccacgtgaagcattggccatggatccgcaacaacgtattatgttggaaatttcgtgggaagcgctggagcgcgctggtcatgaccctgtgagtttgcgcgggagtgcgaccggggtgttcaccggagtggggaccgtggactatggcccccgtccagatgaagcacctgacgaagttttaggttatgtgggcacgggaactgctagcagtgtagcctcggggcgcgtggcgtattgcctgggacttgagggcccagccatgactgtagataagagacccta

SEQ ID NO: 30 - DNA, 1169 bp, Artificial Sequence
  DNA fragment
tagggtctcatctggcgagtggggaaactgcagtcgtggtaactgacgtcgactggccggcgttcgccgaatcatacaccgcggcacgcccgcgtcctctgttagatcgcattgtgaccaccgcaccatcagagcgtgcgggtgagccagaaacggaatcgcttcgcgatcgtctcgctggattaccacgcgctgagcgcaccgcggaactggtacgcttagtacgtactagtaccgcgaccgtcttgggccacgatgatccaaaggcggtccgcgccacgaccccgtttaaagaattaggcttcgatagcttagccgctgttcgtttacgcaacttactcaatgcagccaccggcctgcgtctgcctagtacgctggtattcgaccacccgaacgcgagtgccgtggctggtttcctggacgccgagcttggtactgaagtgcgtggcgaggctccatcggctctggccggacttgatgcactggaagcggcccttcctgaggtacctgccaccgaacgtgaagagctggtgcaacgcttagaacgtatgttagcggctttacgtccagtcgcgcaggctgccgacgccagcggtacaggcgcgaatccgagcggagatgatctgggtgaagcaggcgttgacgagctccttgaggccctcggccgcgagttagacggggactagtagcataaccccttggggcctctaaacgggtcttgaggggttttttgactacgagatttgaggtaatctccgcttctagtacctcactaatacgactcactatagggagaagctgtcaccggatgtgctttccggtctgatgagtccgtgaggacgaaacagcctctacaaataattttgtttaatttgtttaactttaagaaggagaatgacagattcagagaaagttgcagagtacttgcgccgcgccacgcttgaccttcgtgccgcgcgccaacgcattcgtgagctggaaagcgatcccattgcgatcgtctcgatggcgtgtcgtctgccgggtggtgtgaacaccccacaacgtttatgggagctgctccgtgagggcggggaaaccttgtcgggctttcccaccgatcgtggctgggaccttgctcgtttgcatcacccggacccggataatccaggaacgtcttagagacccta

SEQ ID NO: 31 - DNA, 780 bp, Artificial Sequence
  DNA fragment
tagggtctcaattatcgagcacctgcttggattaccgtggttgtctccgcttctagtacctcactaatacgactcactatagggagaagctgtcaccggatgtgctttccggtctgatgagtccgtgaggacgaaacagcctctacaaataattttgtttaatttgtttaactttaagaaggagaatggccgacttatcgaaactgtcagattcgcgtaccgcccaacccggccgcattgtgcgcccttggccacttagtggttgtaacgaatctgcccttcgtgcccgcgcgcgccaactgcgtgcccacttagaccgctttccggacgccggcgtggaaggcgtgggtgcagcgctggcacatgatgaacaagcagatgcaggcccccatcgtgctgttgtggtggcaagctctactagcgaactgttagacggtctggcggccgtggcggatgggcgcccacatgcctcagtagttcgtggcgtagctcgcccgtcagcacctgttgttttcgtatttccgggtcaaggagcccaatgggcgggcatggccggtgagttgctgggtgagtcccgcgtgttcgcagcggcgatggatgcttgcgcacgtgccttcgaacccgtgacagattggaccctcgcgcaagtactggattcaccggaacaaagtcgccgcgtagaagtagtacagccggcgctgttcgcagtgcagacgagcctcgcagccttatggcgcagtttcggggtgacgccagacgccgtggttggccactccattg